European Patent Application EP 4 647 124 A2, published November 12, 2025. Title: Therapeutics for the treatment of neurodegenerative disorders. Applicant: UCL Business Ltd. Application US 18/920273, filed February 13, 2025. The sequence listing filed with the application follows.

SEQUENCE LISTING (583 sequences)

SEQ ID NO: 1 - RNA, 1288 nt, Homo sapiens
  misc_feature 414: note = G can be replaced with C at this position
  misc_feature 964: note = U can be replaced with G at this position
  source 1..1288: mol_type = other RNA
gtgagggtcattgctcggcccctcccatgccacttccactcaccattcctgcctgcccagctcttcctctttctggccacaccatccacactctcctggccctctgagactgcccgccatgccattccctttacctggaaaactcctccctatccatcaaagtccagattcagggtcacctcctctgggaagcccaccttggcctccaggttgactctcactactcatcatcaggttcttccttctattccagccctaaccactcaggattgggccgtttgtgtctgggtatgtctcttccagctgcctgggtttcctggaaagaactcttatccccaggaactagtttgttgaataaatgctggtgaatgaatgaatgattgaacagatgaatgagtgatgagtagataaaaggatggatggagagatgggtgagtacatggatggatagatggatgagttggtgggtagattcgtggctagatggatgatggatggatggacagatggatggatatatgattgaactattgaaagtatagatgtatggatgggtgaatttgggggtaattgttagatgatggatgagtatagatgaatgatggatggataacttgatgagtggatagatagattgctggatagatgattgactgggtggatagatgaaatgttggatgagcagattaagttgtattggatgggatggatggaagtgtggttgagttattagaaggaagattgagtagataggtgaatttgttgatagtcagatgggtagataggtagatggatggatggatggatggatgtataggcagatggacaaatggatgaatgggtgggtggatgaatggaaggatgtgtggttgaactattgcaagtattgataattgggttcataatttctgaatatttagatggatggttgtgagtggctggtggacagacgaaaaatggatggttggataaattgatgggtggatggatggttggttgtatgaaagaatgaatgattgggtaggtggattaagttgcggatcaatgtatgggatggatgaatggatggatggatggatgtgtggttgaattactgaaaggttggaagagtggatgggtgaaatttggggtagttagatgggtgggtgtgtggatggataaaagagtagatgaatgaattaatgaataaacaggcagatggatgatgtaagctgccccagaccctgggacctctgacccccggcgaccccttgcactctccatgacactttctctcccatggtggcag

SEQ ID NO: 2 - RNA, 128 nt, Homo sapiens
  misc_feature 112: note = G can be replaced with C at this position
  source 1..128: mol_type = other RNA
ctgcctgggtttcctggaaagaactcttatccccaggaactagtttgttgaataaatgctggtgaatgaatgaatgattgaacagatgaatgagtgatgagtagataaaaggatggatggagagatgg

SEQ ID NO: 3 - RNA, 178 nt, Homo sapiens
  misc_feature 162: note = G at this position can be replaced with C
  source 1..178: mol_type = other RNA
ccctaaccactcaggattgggccgtttgtgtctgggtatgtctcttccagctgcctgggtttcctggaaagaactcttatccccaggaactagtttgttgaataaatgctggtgaatgaatgaatgattgaacagatgaatgagtgatgagtagataaaaggatggatggagagatgg

SEQ ID NO: 4 - RNA, 13 nt, synthetic construct
  misc_feature 1..13: note = Synthetic sequence
  misc_feature 1..13: note = U can be replaced with T
  misc_feature 1..13: note = U can be replaced by T. Any base can be replaced with a modified base.
  source 1..13: mol_type = other RNA
ggagttttccagg

SEQ ID NO: 5 - RNA, 13 nt, synthetic construct
  misc_feature 1..13: note = Synthetic sequence
  misc_feature 1..13: note = U can be replaced by T. Any base can be replaced with a modified base.
  source 1..13: mol_type = other RNA
aggagttttccag

SEQ ID NO: 6 - RNA, 13 nt, synthetic construct
  misc_feature 1..13: note = Synthetic sequence
  misc_feature 1..13: note = U can be replaced by T. Any base can be replaced with a modified base.
  source 1..13: mol_type = other RNA
gaggagttttcca

SEQ ID NO: 7 - RNA, 13 nt, synthetic construct
  misc_feature 1..13: note = Synthetic sequence
  misc_feature 1..13: note = U can be replaced by T. Any base can be replaced with a modified base.
  source 1..13: mol_type = other RNA
ggaggagttttcc

SEQ ID NO: 8 - RNA, 13 nt, synthetic construct
  misc_feature 1..13: note = Synthetic sequence
  misc_feature 1..13: note = U can be replaced by T. Any base can be replaced with a modified base.
  source 1..13: mol_type = other RNA
gggaggagttttc

SEQ ID NO: 9 - RNA, 13 nt, synthetic construct
  misc_feature 1..13: note = Synthetic sequence
  misc_feature 1..13: note = U can be replaced by T. Any base can be replaced with a modified base.
  source 1..13: mol_type = other RNA
agggaggagtttt

SEQ ID NO: 10 - RNA, 13 nt, synthetic construct
  misc_feature 1..13: note = Synthetic sequence
  misc_feature 1..13: note = U can be replaced by T. Any base can be replaced with a modified base.
  source 1..13: mol_type = other RNA
tagggaggagttt

SEQ ID NO: 11 - RNA, 13 nt, synthetic construct
  misc_feature 1..13: note = Synthetic sequence
  misc_feature 1..13: note = U can be replaced by T. Any base can be replaced with a modified base.
  source 1..13: mol_type = other RNA
atagggaggagtt

SEQ ID NO: 12 - RNA, 13 nt, synthetic construct
  misc_feature 1..13: note = Synthetic sequence
  misc_feature 1..13: note = U can be replaced by T. Any base can be replaced with a modified base.
  source 1..13: mol_type = other RNA
gatagggaggagt

SEQ ID NO: 13 - RNA, 13 nt, synthetic construct
  misc_feature 1..13: note = Synthetic sequence
  misc_feature 1..13: note = U can be replaced by T. Any base can be replaced with a modified base.
  source 1..13: mol_type = other RNA
ggatagggaggag

SEQ ID NO: 14 - RNA, 13 nt, synthetic construct
  misc_feature 1..13: note = Synthetic sequence
  misc_feature 1..13: note = U can be replaced by T. Any base can be replaced with a modified base.
  source 1..13: mol_type = other RNA
tggatagggagga

SEQ ID NO: 15 - RNA, 13 nt, synthetic construct
  misc_feature 1..13: note = Synthetic sequence
  misc_feature 1..13: note = U can be replaced by T. Any base can be replaced with a modified base.
  source 1..13: mol_type = other RNA
atggatagggagg

SEQ ID NO: 16 - RNA, 13 nt, synthetic construct
  misc_feature 1..13: note = Synthetic sequence
  misc_feature 1..13: note = U can be replaced by T. Any base can be replaced with a modified base.
  source 1..13: mol_type = other RNA
gatggatagggag

SEQ ID NO: 17 - RNA, 13 nt, synthetic construct
  misc_feature 1..13: note = Synthetic sequence
  misc_feature 1..13: note = U can be replaced by T. Any base can be replaced with a modified base.
  source 1..13: mol_type = other RNA
tgatggataggga

SEQ ID NO: 18 - RNA, 13 nt, synthetic construct
  misc_feature 1..13: note = Synthetic sequence
  misc_feature 1..13: note = U can be replaced by T. Any base can be replaced with a modified base.
  source 1..13: mol_type = other RNA
ttgatggataggg

SEQ ID NO: 19 - RNA, 13 nt, synthetic construct
  misc_feature 1..13: note = Synthetic sequence
  misc_feature 1..13: note = U can be replaced by T. Any base can be replaced with a modified base.
  source 1..13: mol_type = other RNA
tttgatggatagg

SEQ ID NO: 20 - RNA, 13 nt, synthetic construct
  misc_feature 1..13: note = Synthetic sequence
  misc_feature 1..13: note = U can be replaced by T. Any base can be replaced with a modified base.
  source 1..13: mol_type = other RNA
ctttgatggatag

SEQ ID NO: 21 - RNA, 13 nt, synthetic construct
  misc_feature 1..13: note = Synthetic sequence
  misc_feature 1..13: note = U can be replaced by T. Any base can be replaced with a modified base.
  source 1..13: mol_type = other RNA
actttgatggata

SEQ ID NO: 22 - RNA, 13 nt, synthetic construct
  misc_feature 1..13: note = Synthetic sequence
  misc_feature 1..13: note = U can be replaced by T. Any base can be replaced with a modified base.
  source 1..13: mol_type = other RNA
gactttgatggat

SEQ ID NO: 23 - RNA, 13 nt, synthetic construct
  misc_feature 1..13: note = Synthetic sequence
  misc_feature 1..13: note = U can be replaced by T. Any base can be replaced with a modified base.
  source 1..13: mol_type = other RNA
ggactttgatgga

SEQ ID NO: 24 - RNA, 13 nt, synthetic construct
  misc_feature 1..13: note = Synthetic sequence
  misc_feature 1..13: note = U can be replaced by T. Any base can be replaced with a modified base.
  source 1..13: mol_type = other RNA
tggactttgatgg

SEQ ID NO: 25 - RNA, 13 nt, synthetic construct
  misc_feature 1..13: note = Synthetic sequence
  misc_feature 1..13: note = U can be replaced by T. Any base can be replaced with a modified base.
  source 1..13: mol_type = other RNA
ctggactttgatg

SEQ ID NO: 26 - RNA, 13 nt, synthetic construct
  misc_feature 1..13: note = Synthetic sequence
  misc_feature 1..13: note = U can be replaced by T. Any base can be replaced with a modified base.
  source 1..13: mol_type = other RNA
tctggactttgat

SEQ ID NO: 27 - RNA, 13 nt, synthetic construct
  misc_feature 1..13: note = Synthetic sequence
  misc_feature 1..13: note = U can be replaced by T. Any base can be replaced with a modified base.
  source 1..13: mol_type = other RNA
atctggactttga

SEQ ID NO: 28 - RNA, 13 nt, synthetic construct
  misc_feature 1..13: note = Synthetic sequence
  misc_feature 1..13: note = U can be replaced by T. Any base can be replaced with a modified base.
  source 1..13: mol_type = other RNA
aatctggactttg

SEQ ID NO: 29 - RNA, 13 nt, synthetic construct
  misc_feature 1..13: note = Synthetic sequence
  misc_feature 1..13: note = U can be replaced by T. Any base can be replaced with a modified base.
  source 1..13: mol_type = other RNA
gaatctggacttt

SEQ ID NO: 30 - RNA, 13 nt, synthetic construct
  misc_feature 1..13: note = Synthetic sequence
  misc_feature 1..13: note = U can be replaced by T. Any base can be replaced with a modified base.
  source 1..13: mol_type = other RNA
tgaatctggactt

SEQ ID NO: 31 - RNA, 13 nt, synthetic construct
  misc_feature 1..13: note = Synthetic sequence
  misc_feature 1..13: note = U can be replaced by T. Any base can be replaced with a modified base.
  source 1..13: mol_type = other RNA
ctgaatctggact

SEQ ID NO: 32 - RNA, 13 nt, synthetic construct
  misc_feature 1..13: note = Synthetic sequence
  misc_feature 1..13: note = U can be replaced by T. Any base can be replaced with a modified base.
  source 1..13: mol_type = other RNA
cctgaatctggac

SEQ ID NO: 33 - RNA, 13 nt, synthetic construct
  misc_feature 1..13: note = Synthetic sequence
  misc_feature 1..13: note = U can be replaced by T. Any base can be replaced with a modified base.
  source 1..13: mol_type = other RNA
ccctgaatctgga

SEQ ID NO: 34 - RNA, 13 nt, synthetic construct
  misc_feature 1..13: note = Synthetic sequence
  misc_feature 1..13: note = U can be replaced by T. Any base can be replaced with a modified base.
  source 1..13: mol_type = other RNA
accctgaatctgg

SEQ ID NO: 35 - RNA, 13 nt, synthetic construct
  misc_feature 1..13: note = Synthetic sequence
  misc_feature 1..13: note = U can be replaced by T. Any base can be replaced with a modified base.
  source 1..13: mol_type = other RNA
gaccctgaatctg

SEQ ID NO: 36 - RNA, 13 nt, synthetic construct
  misc_feature 1..13: note = Synthetic sequence
  misc_feature 1..13: note = U can be replaced by T. Any base can be replaced with a modified base.
  source 1..13: mol_type = other RNA
tgaccctgaatct

SEQ ID NO: 37 - RNA, 13 nt, synthetic construct
  misc_feature 1..13: note = Synthetic sequence
  misc_feature 1..13: note = U can be replaced by T. Any base can be replaced with a modified base.
  source 1..13: mol_type = other RNA
gtgaccctgaatc

SEQ ID NO: 38 - RNA, 13 nt, synthetic construct
  misc_feature 1..13: note = Synthetic sequence
  misc_feature 1..13: note = U can be replaced by T. Any base can be replaced with a modified base.
  source 1..13: mol_type = other RNA
ggtgaccctgaat

SEQ ID NO: 39 - RNA, 13 nt, synthetic construct
  misc_feature 1..13: note = Synthetic sequence
  misc_feature 1..13: note = U can be replaced by T. Any base can be replaced with a modified base.
  source 1..13: mol_type = other RNA
aggtgaccctgaa

SEQ ID NO: 40 - RNA, 13 nt, synthetic construct
  misc_feature 1..13: note = Synthetic sequence
  misc_feature 1..13: note = U can be replaced by T. Any base can be replaced with a modified base.
  source 1..13: mol_type = other RNA
gaggtgaccctga

SEQ ID NO: 41 - RNA, 13 nt, synthetic construct
  misc_feature 1..13: note = Synthetic sequence
  misc_feature 1..13: note = U can be replaced by T. Any base can be replaced with a modified base.
  source 1..13: mol_type = other RNA
ggaggtgaccctg

SEQ ID NO: 42 - RNA, 13 nt, synthetic construct
  misc_feature 1..13: note = Synthetic sequence
  misc_feature 1..13: note = U can be replaced by T. Any base can be replaced with a modified base.
  source 1..13: mol_type = other RNA
aggaggtgaccct

SEQ ID NO: 43 - RNA, 13 nt, synthetic construct
  misc_feature 1..13: note = Synthetic sequence
  misc_feature 1..13: note = U can be replaced by T. Any base can be replaced with a modified base.
  source 1..13: mol_type = other RNA
gaggaggtgaccc

SEQ ID NO: 44 - RNA, 13 nt, synthetic construct
  misc_feature 1..13: note = Synthetic sequence
  misc_feature 1..13: note = U can be replaced by T. Any base can be replaced with a modified base.
  source 1..13: mol_type = other RNA
agaggaggtgacc

SEQ ID NO: 45 - RNA, 13 nt, synthetic construct
  misc_feature 1..13: note = Synthetic sequence
  misc_feature 1..13: note = U can be replaced by T. Any base can be replaced with a modified base.
  source 1..13: mol_type = other RNA
cagaggaggtgac

SEQ ID NO: 46 - RNA, 13 nt, synthetic construct
  misc_feature 1..13: note = Synthetic sequence
  misc_feature 1..13: note = U can be replaced by T. Any base can be replaced with a modified base.
  source 1..13: mol_type = other RNA
ccagaggaggtga

SEQ ID NO: 47 - RNA, 13 nt, synthetic construct
  misc_feature 1..13: note = Synthetic sequence
  misc_feature 1..13: note = U can be replaced by T. Any base can be replaced with a modified base.
  source 1..13: mol_type = other RNA
cccagaggaggtg

SEQ ID NO: 48 - RNA, 13 nt, synthetic construct
  misc_feature 1..13: note = Synthetic sequence
  misc_feature 1..13: note = U can be replaced by T. Any base can be replaced with a modified base.
  source 1..13: mol_type = other RNA
tcccagaggaggt

SEQ ID NO: 49 - RNA, 13 nt, synthetic construct
  misc_feature 1..13: note = Synthetic sequence
  misc_feature 1..13: note = U can be replaced by T. Any base can be replaced with a modified base.
  source 1..13: mol_type = other RNA
ttcccagaggagg

SEQ ID NO: 50 - RNA, 13 nt, synthetic construct
  misc_feature 1..13: note = Synthetic sequence
  misc_feature 1..13: note = U can be replaced by T. Any base can be replaced with a modified base.
  source 1..13: mol_type = other RNA
cttcccagaggag

SEQ ID NO: 51 - RNA, 13 nt, synthetic construct
  misc_feature 1..13: note = Synthetic sequence
  misc_feature 1..13: note = U can be replaced by T. Any base can be replaced with a modified base.
  source 1..13: mol_type = other RNA
gcttcccagagga

SEQ ID NO: 52 - RNA, 13 nt, synthetic construct
  misc_feature 1..13: note = Synthetic sequence
  misc_feature 1..13: note = U can be replaced by T. Any base can be replaced with a modified base.
  source 1..13: mol_type = other RNA
ggcttcccagagg

SEQ ID NO: 53 - RNA, 13 nt, synthetic construct
  misc_feature 1..13: note = Synthetic sequence
  misc_feature 1..13: note = U can be replaced by T. Any base can be replaced with a modified base.
  source 1..13: mol_type = other RNA
gggcttcccagag

SEQ ID NO: 54 - RNA, 13 nt, synthetic construct
  misc_feature 1..13: note = Synthetic sequence
  misc_feature 1..13: note = U can be replaced by T. Any base can be replaced with a modified base.
  source 1..13: mol_type = other RNA
tgggcttcccaga

SEQ ID NO: 55 - RNA, 13 nt, synthetic construct
  misc_feature 1..13: note = Synthetic sequence
  misc_feature 1..13: note = U can be replaced by T. Any base can be replaced with a modified base.
  source 1..13: mol_type = other RNA
gtgggcttcccag

SEQ ID NO: 56 - RNA, 13 nt, synthetic construct
  misc_feature 1..13: note = Synthetic sequence
  misc_feature 1..13: note = U can be replaced by T. Any base can be replaced with a modified base.
  source 1..13: mol_type = other RNA
ggtgggcttccca

SEQ ID NO: 57 - RNA, 13 nt, synthetic construct
  misc_feature 1..13: note = Synthetic sequence
  misc_feature 1..13: note = U can be replaced by T. Any base can be replaced with a modified base.
  source 1..13: mol_type = other RNA
aggtgggcttccc

SEQ ID NO: 58 - RNA, 13 nt, synthetic construct
  misc_feature 1..13: note = Synthetic sequence
  misc_feature 1..13: note = U can be replaced by T. Any base can be replaced with a modified base.
  source 1..13: mol_type = other RNA
aaggtgggcttcc

SEQ ID NO: 59 - RNA, 13 nt, synthetic construct
  misc_feature 1..13: note = Synthetic sequence
  misc_feature 1..13: note = U can be replaced by T. Any base can be replaced with a modified base.
  source 1..13: mol_type = other RNA
caaggtgggcttc

SEQ ID NO: 60 - RNA, 13 nt, synthetic construct
  misc_feature 1..13: note = Synthetic sequence
  misc_feature 1..13: note = U can be replaced by T. Any base can be replaced with a modified base.
  source 1..13: mol_type = other RNA
ccaaggtgggctt

SEQ ID NO: 61 - RNA, 13 nt, synthetic construct
  misc_feature 1..13: note = Synthetic sequence
  misc_feature 1..13: note = U can be replaced by T. Any base can be replaced with a modified base.
  source 1..13: mol_type = other RNA
gccaaggtgggct

SEQ ID NO: 62 - RNA, 13 nt, synthetic construct
  misc_feature 1..13: note = Synthetic sequence
  misc_feature 1..13: note = U can be replaced by T. Any base can be replaced with a modified base.
  source 1..13: mol_type = other RNA
ggccaaggtgggc

SEQ ID NO: 63 - RNA, 13 nt, synthetic construct
  misc_feature 1..13: note = Synthetic sequence
  misc_feature 1..13: note = U can be replaced by T. Any base can be replaced with a modified base.
  source 1..13: mol_type = other RNA
aggccaaggtggg

SEQ ID NO: 64 - RNA, 13 nt, synthetic construct
  misc_feature 1..13: note = Synthetic sequence
  misc_feature 1..13: note = U can be replaced by T. Any base can be replaced with a modified base.
  source 1..13: mol_type = other RNA
gaggccaaggtgg

SEQ ID NO: 65 - RNA, 13 nt, synthetic construct
  misc_feature 1..13: note = Synthetic sequence
  misc_feature 1..13: note = U can be replaced by T. Any base can be replaced with a modified base.
  source 1..13: mol_type = other RNA
ggaggccaaggtg

SEQ ID NO: 66 - RNA, 13 nt, synthetic construct
  misc_feature 1..13: note = Synthetic sequence
  misc_feature 1..13: note = U can be replaced by T. Any base can be replaced with a modified base.
  source 1..13: mol_type = other RNA
tggaggccaaggt

SEQ ID NO: 67 - RNA, 13 nt, synthetic construct
  misc_feature 1..13: note = Synthetic sequence
  misc_feature 1..13: note = U can be replaced by T. Any base can be replaced with a modified base.
  source 1..13: mol_type = other RNA
ctggaggccaagg

SEQ ID NO: 68 - RNA, 13 nt, synthetic construct
  misc_feature 1..13: note = Synthetic sequence
  misc_feature 1..13: note = U can be replaced by T. Any base can be replaced with a modified base.
  source 1..13: mol_type = other RNA
cctggaggccaag

SEQ ID NO: 69 - RNA, 13 nt, synthetic construct
  misc_feature 1..13: note = Synthetic sequence
  misc_feature 1..13: note = U can be replaced by T. Any base can be replaced with a modified base.
  source 1..13: mol_type = other RNA
acctggaggccaa

SEQ ID NO: 70 - RNA, 13 nt, synthetic construct
  misc_feature 1..13: note = Synthetic sequence
  misc_feature 1..13: note = U can be replaced by T. Any base can be replaced with a modified base.
  source 1..13: mol_type = other RNA
aacctggaggcca

SEQ ID NO: 71 - RNA, 13 nt, synthetic construct
  misc_feature 1..13: note = Synthetic sequence
  misc_feature 1..13: note = U can be replaced by T. Any base can be replaced with a modified base.
  source 1..13: mol_type = other RNA
caacctggaggcc

SEQ ID NO: 72 - RNA, 13 nt, synthetic construct
  misc_feature 1..13: note = Synthetic sequence
  misc_feature 1..13: note = U can be replaced by T. Any base can be replaced with a modified base.
  source 1..13: mol_type = other RNA
tcaacctggaggc

SEQ ID NO: 73 - RNA, 13 nt, synthetic construct
  misc_feature 1..13: note = Synthetic sequence
  misc_feature 1..13: note = U can be replaced by T. Any base can be replaced with a modified base.
  source 1..13: mol_type = other RNA
gtcaacctggagg

SEQ ID NO: 74 - RNA, 13 nt, synthetic construct
  misc_feature 1..13: note = Synthetic sequence
  misc_feature 1..13: note = U can be replaced by T. Any base can be replaced with a modified base.
  source 1..13: mol_type = other RNA
agtcaacctggag

SEQ ID NO: 75 - RNA, 13 nt, synthetic construct
  misc_feature 1..13: note = Synthetic sequence
  misc_feature 1..13: note = U can be replaced by T. Any base can be replaced with a modified base.
  source 1..13: mol_type = other RNA
gagtcaacctgga

SEQ ID NO: 76 - RNA, 13 nt, synthetic construct
  misc_feature 1..13: note = Synthetic sequence
  misc_feature 1..13: note = U can be replaced by T. Any base can be replaced with a modified base.
  source 1..13: mol_type = other RNA
agagtcaacctgg

SEQ ID NO: 77 - RNA, 13 nt, synthetic construct
  misc_feature 1..13: note = Synthetic sequence
  misc_feature 1..13: note = U can be replaced by T. Any base can be replaced with a modified base.
  source 1..13: mol_type = other RNA
gagagtcaacctg

SEQ ID NO: 78 - RNA, 13 nt, synthetic construct
  misc_feature 1..13: note = Synthetic sequence
  misc_feature 1..13: note = U can be replaced by T. Any base can be replaced with a modified base.
  source 1..13: mol_type = other RNA
tgagagtcaacct

SEQ ID NO: 79 - RNA, 13 nt, synthetic construct
  misc_feature 1..13: note = Synthetic sequence
  misc_feature 1..13: note = U can be replaced by T. Any base can be replaced with a modified base.
  source 1..13: mol_type = other RNA
gtgagagtcaacc

SEQ ID NO: 80 - RNA, 13 nt, synthetic construct
  misc_feature 1..13: note = Synthetic sequence
  misc_feature 1..13: note = U can be replaced by T. Any base can be replaced with a modified base.
  source 1..13: mol_type = other RNA
agtgagagtcaac

SEQ ID NO: 81 - RNA, 13 nt, synthetic construct
  misc_feature 1..13: note = Synthetic sequence
  misc_feature 1..13: note = U can be replaced by T. Any base can be replaced with a modified base.
  source 1..13: mol_type = other RNA
tagtgagagtcaa

SEQ ID NO: 82 - RNA, 13 nt, synthetic construct
  misc_feature 1..13: note = Synthetic sequence
  misc_feature 1..13: note = U can be replaced by T. Any base can be replaced with a modified base.
  source 1..13: mol_type = other RNA
gtagtgagagtca

SEQ ID NO: 83 - RNA, 13 nt, synthetic construct
  misc_feature 1..13: note = Synthetic sequence
  misc_feature 1..13: note = U can be replaced by T. Any base can be replaced with a modified base.
  source 1..13: mol_type = other RNA
agtagtgagagtc

SEQ ID NO: 84 - RNA, 13 nt, synthetic construct
  misc_feature 1..13: note = Synthetic sequence
  misc_feature 1..13: note = U can be replaced by T. Any base can be replaced with a modified base.
  source 1..13: mol_type = other RNA
gagtagtgagagt

SEQ ID NO: 85 - RNA, 13 nt, synthetic construct
  misc_feature 1..13: note = Synthetic sequence
  misc_feature 1..13: note = U can be replaced by T. Any base can be replaced with a modified base.
  source 1..13: mol_type = other RNA
tgagtagtgagag

SEQ ID NO: 86 - RNA, 13 nt, synthetic construct
  misc_feature 1..13: note = Synthetic sequence
  misc_feature 1..13: note = U can be replaced by T. Any base can be replaced with a modified base.
  source 1..13: mol_type = other RNA
atgagtagtgaga

SEQ ID NO: 87 - RNA, 13 nt, synthetic construct
  misc_feature 1..13: note = Synthetic sequence
  misc_feature 1..13: note = U can be replaced by T. Any base can be replaced with a modified base.
  source 1..13: mol_type = other RNA
gatgagtagtgag

SEQ ID NO: 88 - RNA, 13 nt, synthetic construct
  misc_feature 1..13: note = Synthetic sequence
  misc_feature 1..13: note = U can be replaced by T. Any base can be replaced with a modified base.
  source 1..13: mol_type = other RNA
tgatgagtagtga

SEQ ID NO: 89 - RNA, 13 nt, synthetic construct
  misc_feature 1..13: note = Synthetic sequence
  misc_feature 1..13: note = U can be replaced by T. Any base can be replaced with a modified base.
  source 1..13: mol_type = other RNA
atgatgagtagtg

SEQ ID NO: 90 - RNA, 13 nt, synthetic construct
  misc_feature 1..13: note = Synthetic sequence
  misc_feature 1..13: note = U can be replaced by T. Any base can be replaced with a modified base.
  source 1..13: mol_type = other RNA
gatgatgagtagt

SEQ ID NO: 91 - RNA, 13 nt, synthetic construct
  misc_feature 1..13: note = Synthetic sequence
  misc_feature 1..13: note = U can be replaced by T. Any base can be replaced with a modified base.
  source 1..13: mol_type = other RNA
tgatgatgagtag

SEQ ID NO: 92 - RNA, 13 nt, synthetic construct
  misc_feature 1..13: note = Synthetic sequence
  misc_feature 1..13: note = U can be replaced by T. Any base can be replaced with a modified base.
  source 1..13: mol_type = other RNA
ctgatgatgagta

SEQ ID NO: 93 - RNA, 13 nt, synthetic construct
  misc_feature 1..13: note = Synthetic sequence
  misc_feature 1..13: note = U can be replaced by T. Any base can be replaced with a modified base.
  source 1..13: mol_type = other RNA
cctgatgatgagt

SEQ ID NO: 94 - RNA, 13 nt, synthetic construct
  misc_feature 1..13: note = Synthetic sequence
  misc_feature 1..13: note = U can be replaced by T. Any base can be replaced with a modified base.
  source 1..13: mol_type = other RNA
acctgatgatgag

SEQ ID NO: 95 - RNA, 13 nt, synthetic construct
  misc_feature 1..13: note = Synthetic sequence
  misc_feature 1..13: note = U can be replaced by T. Any base can be replaced with a modified base.
  source 1..13: mol_type = other RNA
aacctgatgatga

SEQ ID NO: 96 - RNA, 13 nt, synthetic construct
  misc_feature 1..13: note = Synthetic sequence
  misc_feature 1..13: note = U can be replaced by T. Any base can be replaced with a modified base.
  source 1..13: mol_type = other RNA
gaacctgatgatg

SEQ ID NO: 97 - RNA, 13 nt, synthetic construct
  misc_feature 1..13: note = Synthetic sequence
  misc_feature 1..13: note = U can be replaced by T. Any base can be replaced with a modified base.
  source 1..13: mol_type = other RNA
agaacctgatgat

SEQ ID NO: 98 - RNA, 13 nt, synthetic construct
  misc_feature 1..13: note = Synthetic sequence
  misc_feature 1..13: note = U can be replaced by T. Any base can be replaced with a modified base.
  source 1..13: mol_type = other RNA
aagaacctgatga

SEQ ID NO: 99 - RNA, 13 nt, synthetic construct
  misc_feature 1..13: note = Synthetic sequence
  misc_feature 1..13: note = U can be replaced by T. Any base can be replaced with a modified base.
  source 1..13: mol_type = other RNA
gaagaacctgatg

SEQ ID NO: 100 - RNA, 13 nt, synthetic construct
  misc_feature 1..13: note = Synthetic sequence
  misc_feature 1..13: note = U can be replaced by T. Any base can be replaced with a modified base.
  source 1..13: mol_type = other RNA
ggaagaacctgat

SEQ ID NO: 101 - RNA, 13 nt, synthetic construct
  misc_feature 1..13: note = Synthetic sequence
  misc_feature 1..13: note = U can be replaced by T. Any base can be replaced with a modified base.
  source 1..13: mol_type = other RNA
aggaagaacctga

SEQ ID NO: 102 - RNA, 13 nt, synthetic construct
  misc_feature 1..13: note = Synthetic sequence
  misc_feature 1..13: note = U can be replaced by T. Any base can be replaced with a modified base.
  source 1..13: mol_type = other RNA
aaggaagaacctg

SEQ ID NO: 103 - RNA, 13 nt, synthetic construct
  misc_feature 1..13: note = Synthetic sequence
  misc_feature 1..13: note = U can be replaced by T. Any base can be replaced with a modified base.
  source 1..13: mol_type = other RNA
gaaggaagaacct

SEQ ID NO: 104 - RNA, 13 nt, synthetic construct
  misc_feature 1..13: note = Synthetic sequence
  misc_feature 1..13: note = U can be replaced by T. Any base can be replaced with a modified base.
  source 1..13: mol_type = other RNA
agaaggaagaacc

SEQ ID NO: 105 - RNA, 13 nt, synthetic construct
  misc_feature 1..13: note = Synthetic sequence
  misc_feature 1..13: note = U can be replaced by T. Any base can be replaced with a modified base.
  source 1..13: mol_type = other RNA
tagaaggaagaac

SEQ ID NO: 106 - RNA, 13 nt, synthetic construct
  misc_feature 1..13: note = Synthetic sequence
  misc_feature 1..13: note = U can be replaced by T. Any base can be replaced with a modified base.
  source 1..13: mol_type = other RNA
atagaaggaagaa

SEQ ID NO: 107 - RNA, 13 nt, synthetic construct
  misc_feature 1..13: note = Synthetic sequence
  misc_feature 1..13: note = U can be replaced by T. Any base can be replaced with a modified base.
  source 1..13: mol_type = other RNA
aatagaaggaaga

SEQ ID NO: 108 - RNA, 13 nt, synthetic construct
  misc_feature 1..13: note = Synthetic sequence
  misc_feature 1..13: note = U can be replaced by T. Any base can be replaced with a modified base.
  source 1..13: mol_type = other RNA
gaatagaaggaag

SEQ ID NO: 109 - RNA, 13 nt, synthetic construct
  misc_feature 1..13: note = Synthetic sequence
  misc_feature 1..13: note = U can be replaced by T. Any base can be replaced with a modified base.
  source 1..13: mol_type = other RNA
ggaatagaaggaa

SEQ ID NO: 110 - RNA, 13 nt, synthetic construct
  misc_feature 1..13: note = Synthetic sequence
  misc_feature 1..13: note = U can be replaced by T. Any base can be replaced with a modified base.
  source 1..13: mol_type = other RNA
tggaatagaagga

SEQ ID NO: 111 - RNA, 13 nt, synthetic construct
  misc_feature 1..13: note = Synthetic sequence
  misc_feature 1..13: note = U can be replaced by T. Any base can be replaced with a modified base.
  source 1..13: mol_type = other RNA
ctggaatagaagg

SEQ ID NO: 112 - RNA, 13 nt, synthetic construct
  misc_feature 1..13: note = Synthetic sequence
  misc_feature 1..13: note = U can be replaced by T. Any base can be replaced with a modified base.
  source 1..13: mol_type = other RNA
gctggaatagaag

SEQ ID NO: 113 - RNA, 13 nt, synthetic construct
  misc_feature 1..13: note = Synthetic sequence
  misc_feature 1..13: note = U can be replaced by T. Any base can be replaced with a modified base.
  source 1..13: mol_type = other RNA
ggctggaatagaa

SEQ ID NO: 114 - RNA, 13 nt, synthetic construct
  misc_feature 1..13: note = Synthetic sequence
  misc_feature 1..13: note = U can be replaced by T. Any base can be replaced with a modified base.
  source 1..13: mol_type = other RNA
gggctggaataga

SEQ ID NO: 115 - RNA, 13 nt, synthetic construct
  misc_feature 1..13: note = Synthetic sequence
  misc_feature 1..13: note = U can be replaced by T. Any base can be replaced with a modified base.
  source 1..13: mol_type = other RNA
agggctggaatag

SEQ ID NO: 116 - RNA, 13 nt, synthetic construct
  misc_feature 1..13: note = Synthetic sequence
  misc_feature 1..13: note = U can be replaced by T. Any base can be replaced with a modified base.
  source 1..13: mol_type = other RNA
tagggctggaata

SEQ ID NO: 117 - RNA, 13 nt, synthetic construct
  misc_feature 1..13: note = Synthetic sequence
  misc_feature 1..13: note = U can be replaced by T. Any base can be replaced with a modified base.
  source 1..13: mol_type = other RNA
ttagggctggaat

SEQ ID NO: 118 - RNA, 13 nt, synthetic construct
  misc_feature 1..13: note = Synthetic sequence
  misc_feature 1..13: note = U can be replaced by T. Any base can be replaced with a modified base.
  source 1..13: mol_type = other RNA
gttagggctggaa

SEQ ID NO: 119 - RNA, 13 nt, synthetic construct
  misc_feature 1..13: note = Synthetic sequence
  misc_feature 1..13: note = U can be replaced by T. Any base can be replaced with a modified base.
  source 1..13: mol_type = other RNA
ggttagggctgga

SEQ ID NO: 120 - RNA, 13 nt, synthetic construct
  misc_feature 1..13: note = Synthetic sequence
  misc_feature 1..13: note = U can be replaced by T. Any base can be replaced with a modified base.
  source 1..13: mol_type = other RNA
tggttagggctgg

SEQ ID NO: 121 - RNA, 13 nt, synthetic construct
  misc_feature 1..13: note = Synthetic sequence
  misc_feature 1..13: note = U can be replaced by T. Any base can be replaced with a modified base.
  source 1..13: mol_type = other RNA
gtggttagggctg

SEQ ID NO: 122 - RNA, 13 nt, synthetic construct
  misc_feature 1..13: note = Synthetic sequence
  misc_feature 1..13: note = U can be replaced by T. Any base can be replaced with a modified base.
  source 1..13: mol_type = other RNA
agtggttagggct

SEQ ID NO: 123 - RNA, 13 nt, synthetic construct
  misc_feature 1..13: note = Synthetic sequence
  misc_feature 1..13: note = U can be replaced by T. Any base can be replaced with a modified base.
  source 1..13: mol_type = other RNA
gagtggttagggc

SEQ ID NO: 124 - RNA, 13 nt, synthetic construct
  misc_feature 1..13: note = Synthetic sequence
  misc_feature 1..13: note = U can be replaced by T. Any base can be replaced with a modified base.
  source 1..13: mol_type = other RNA
tgagtggttaggg

SEQ ID NO: 125 - RNA, 13 nt, synthetic construct
  misc_feature 1..13: note = Synthetic sequence
  misc_feature 1..13: note = U can be replaced by T. Any base can be replaced with a modified base.
  source 1..13: mol_type = other RNA
ctgagtggttagg

SEQ ID NO: 126 - RNA, 13 nt, synthetic construct
  misc_feature 1..13: note = Synthetic sequence
  misc_feature 1..13: note = U can be replaced by T. Any base can be replaced with a modified base.
  source 1..13: mol_type = other RNA
cctgagtggttag

SEQ ID NO: 127 - RNA, 13 nt, synthetic construct
  misc_feature 1..13: note = Synthetic sequence
  misc_feature 1..13: note = U can be replaced by T. Any base can be replaced with a modified base.
  source 1..13: mol_type = other RNA
tcctgagtggtta

SEQ ID NO: 128 - RNA, 13 nt, synthetic construct
  misc_feature 1..13: note = Synthetic sequence
  misc_feature 1..13: note = U can be replaced by T. Any base can be replaced with a modified base.
  source 1..13: mol_type = other RNA
atcctgagtggtt

SEQ ID NO: 129 - RNA, 13 nt, synthetic construct
  misc_feature 1..13: note = Synthetic sequence
  misc_feature 1..13: note = U can be replaced by T. Any base can be replaced with a modified base.
  source 1..13: mol_type = other RNA
aatcctgagtggt

SEQ ID NO: 130 - RNA, 13 nt, synthetic construct
  misc_feature 1..13: note = Synthetic sequence
  misc_feature 1..13: note = U can be replaced by T. Any base can be replaced with a modified base.
  source 1..13: mol_type = other RNA
caatcctgagtgg

SEQ ID NO: 131 - RNA, 13 nt, synthetic construct
  misc_feature 1..13: note = Synthetic sequence
  misc_feature 1..13: note = U can be replaced by T. Any base can be replaced with a modified base.
  source 1..13: mol_type = other RNA
ccaatcctgagtg

SEQ ID NO: 132 - RNA, 13 nt, synthetic construct
  misc_feature 1..13: note = Synthetic sequence
  misc_feature 1..13: note = U can be replaced by T. Any base can be replaced with a modified base.
  source 1..13: mol_type = other RNA
cccaatcctgagt

SEQ ID NO: 133 - RNA, 13 nt, synthetic construct
  misc_feature 1..13: note = Synthetic sequence
  misc_feature 1..13: note = U can be replaced by T. Any base can be replaced with a modified base.
  source 1..13: mol_type = other RNA
gcccaatcctgag

SEQ ID NO: 134 - RNA, 13 nt, synthetic construct
  misc_feature 1..13: note = Synthetic sequence
  misc_feature 1..13: note = U can be replaced by T. Any base can be replaced with a modified base.
  source 1..13: mol_type = other RNA
ggcccaatcctga

SEQ ID NO: 135 - RNA, 13 nt, synthetic construct
  misc_feature 1..13: note = Synthetic sequence
  misc_feature 1..13: note = U can be replaced by T. Any base can be replaced with a modified base.
  source 1..13: mol_type = other RNA
cggcccaatcctg

SEQ ID NO: 136 - RNA, 13 nt, synthetic construct
  misc_feature 1..13: note = Synthetic sequence
  misc_feature 1..13: note = U can be replaced by T. Any base can be replaced with a modified base.
  source 1..13: mol_type = other RNA
acggcccaatcct

SEQ ID NO: 137 - RNA, 13 nt, synthetic construct
  misc_feature 1..13: note = Synthetic sequence
  misc_feature 1..13: note = U can be replaced by T. Any base can be replaced with a modified base.
  source 1..13: mol_type = other RNA
aacggcccaatcc

SEQ ID NO: 138 - RNA, 13 nt, synthetic construct
  misc_feature 1..13: note = Synthetic sequence
  misc_feature 1..13: note = U can be replaced by T. Any base can be replaced with a modified base.
  source 1..13: mol_type = other RNA
aaacggcccaatc

SEQ ID NO: 139 - RNA, 13 nt, synthetic construct
  misc_feature 1..13: note = Synthetic sequence
  misc_feature 1..13: note = U can be replaced by T. Any base can be replaced with a modified base.
  source 1..13: mol_type = other RNA
caaacggcccaat

SEQ ID NO: 140 - RNA, 13 nt, synthetic construct
  misc_feature 1..13: note = Synthetic sequence
  misc_feature 1..13: note = U can be replaced by T. Any base can be replaced with a modified base.
  source 1..13: mol_type = other RNA
acaaacggcccaa

SEQ ID NO: 141 - RNA, 13 nt, synthetic construct
  misc_feature 1..13: note = Synthetic sequence
  misc_feature 1..13: note = U can be replaced by T. Any base can be replaced with a modified base.
  source 1..13: mol_type = other RNA
cacaaacggccca

SEQ ID NO: 142 - RNA, 13 nt, synthetic construct
  misc_feature 1..13: note = Synthetic sequence
  misc_feature 1..13: note = U can be replaced by T. Any base can be replaced with a modified base.
  source 1..13: mol_type = other RNA
acacaaacggccc

SEQ ID NO: 143 - RNA, 13 nt, synthetic construct
  misc_feature 1..13: note = Synthetic sequence
  misc_feature 1..13: note = U can be replaced by T. Any base can be replaced with a modified base.
  source 1..13: mol_type = other RNA
gacacaaacggcc

SEQ ID NO: 144 - RNA, 13 nt, synthetic construct
  misc_feature 1..13: note = Synthetic sequence
  misc_feature 1..13: note = U can be replaced by T. Any base can be replaced with a modified base.
  source 1..13: mol_type = other RNA
agacacaaacggc

SEQ ID NO: 145 - RNA, 13 nt, synthetic construct
  misc_feature 1..13: note = Synthetic sequence
  misc_feature 1..13: note = U can be replaced by T. Any base can be replaced with a modified base.
  source 1..13: mol_type = other RNA
cagacacaaacgg

SEQ ID NO: 146 - RNA, 13 nt, synthetic construct
  misc_feature 1..13: note = Synthetic sequence
  misc_feature 1..13: note = U can be replaced by T. Any base can be replaced with a modified base.
  source 1..13: mol_type = other RNA
ccagacacaaacg

SEQ ID NO: 147 - RNA, 13 nt, synthetic construct
  misc_feature 1..13: note = Synthetic sequence
  misc_feature 1..13: note = U can be replaced by T. Any base can be replaced with a modified base.
  source 1..13: mol_type = other RNA
cccagacacaaac

SEQ ID NO: 148 - RNA, 13 nt, synthetic construct
  misc_feature 1..13: note = Synthetic sequence
  misc_feature 1..13: note = U can be replaced by T. Any base can be replaced with a modified base.
  source 1..13: mol_type = other RNA
acccagacacaaa

SEQ ID NO: 149 - RNA, 13 nt, synthetic construct
  misc_feature 1..13: note = Synthetic sequence
  misc_feature 1..13: note = U can be replaced by T. Any base can be replaced with a modified base.
  source 1..13: mol_type = other RNA
tacccagacacaa

SEQ ID NO: 150 - RNA, 13 nt, synthetic construct
  misc_feature 1..13: note = Synthetic sequence
  misc_feature 1..13: note = U can be replaced by T. Any base can be replaced with a modified base.
  source 1..13: mol_type = other RNA
atacccagacaca

SEQ ID NO: 151 - RNA, 13 nt, synthetic construct
  misc_feature 1..13: note = Synthetic sequence
  misc_feature 1..13: note = U can be replaced by T. Any base can be replaced with a modified base.
  source 1..13: mol_type = other RNA
catacccagacac

SEQ ID NO: 152 - RNA, 13 nt, synthetic construct
  misc_feature 1..13: note = Synthetic sequence
  misc_feature 1..13: note = U can be replaced by T. Any base can be replaced with a modified base.
  source 1..13: mol_type = other RNA
acatacccagaca

SEQ ID NO: 153 - RNA, 13 nt, synthetic construct
  misc_feature 1..13: note = Synthetic sequence
  misc_feature 1..13: note = U can be replaced by T. Any base can be replaced with a modified base.
  source 1..13: mol_type = other RNA
gacatacccagac

SEQ ID NO: 154 - RNA, 13 nt, synthetic construct
  misc_feature 1..13: note = Synthetic sequence
  misc_feature 1..13: note = U can be replaced by T. Any base can be replaced with a modified base.
  source 1..13: mol_type = other RNA
agacatacccaga

SEQ ID NO: 155 - RNA, 13 nt, synthetic construct
  misc_feature 1..13: note = Synthetic sequence
  misc_feature 1..13: note = U can be replaced by T. Any base can be replaced with a modified base.
  source 1..13: mol_type = other RNA
gagacatacccag

SEQ ID NO: 156 - RNA, 13 nt, synthetic construct
  misc_feature 1..13: note = Synthetic sequence
  misc_feature 1..13: note = U can be replaced by T. Any base can be replaced with a modified base.
  source 1..13: mol_type = other RNA
agagacataccca

SEQ ID NO: 157 - RNA, 13 nt, synthetic construct
  misc_feature 1..13: note = Synthetic sequence
  misc_feature 1..13: note = U can be replaced by T. Any base can be replaced with a modified base.
  source 1..13: mol_type = other RNA
aagagacataccc

SEQ ID NO: 158 - RNA, 13 nt, synthetic construct
  misc_feature 1..13: note = Synthetic sequence
  misc_feature 1..13: note = U can be replaced by T. Any base can be replaced with a modified base.
  source 1..13: mol_type = other RNA
gaagagacatacc

SEQ ID NO: 159 - RNA, 13 nt, synthetic construct
  misc_feature 1..13: note = Synthetic sequence
  misc_feature 1..13: note = U can be replaced by T. Any base can be replaced with a modified base.
  source 1..13: mol_type = other RNA
ggaagagacatac

SEQ ID NO: 160 - RNA, 13 nt, synthetic construct
  misc_feature 1..13: note = Synthetic sequence
  misc_feature 1..13: note = U can be replaced by T. Any base can be replaced with a modified base.
  source 1..13: mol_type = other RNA
tggaagagacata

SEQ ID NO: 161 - RNA, 13 nt, synthetic construct
  misc_feature 1..13: note = Synthetic sequence
  misc_feature 1..13: note = U can be replaced by T. Any base can be replaced with a modified base.
  source 1..13: mol_type = other RNA
ctggaagagacat

SEQ ID NO: 162 - RNA, 13 nt, synthetic construct
  misc_feature 1..13: note = Synthetic sequence
  misc_feature 1..13: note = U can be replaced by T. Any base can be replaced with a modified base.
  source 1..13: mol_type = other RNA
gctggaagagaca

SEQ ID NO: 163 - RNA, 13 nt, synthetic construct
  misc_feature 1..13: note = Synthetic sequence
  misc_feature 1..13: note = U can be replaced by T. Any base can be replaced with a modified base.
  source 1..13: mol_type = other RNA
agctggaagagac

SEQ ID NO: 164 - RNA, 13 nt, synthetic construct
  misc_feature 1..13: note = Synthetic sequence
  source 1..13: mol_type = other RNA
cagctggaagaga

SEQ ID NO: 165 - RNA, 13 nt, synthetic construct
  misc_feature 1..13: note = Synthetic sequence
  misc_feature 1..13: note = U can be replaced by T. Any base can be replaced with a modified base.
  source 1..13: mol_type = other RNA
gcagctggaagag

SEQ ID NO: 166 - RNA, 13 nt, synthetic construct
  misc_feature 1..13: note = Synthetic sequence
  misc_feature 1..13: note = U can be replaced by T. Any base can be replaced with a modified base.
  source 1..13: mol_type = other RNA
ggcagctggaaga

SEQ ID NO: 167 - RNA, 13 nt, synthetic construct
  misc_feature 1..13: note = Synthetic sequence
  misc_feature 1..13: note = U can be replaced by T. Any base can be replaced with a modified base.
  source 1..13: mol_type = other RNA
aggcagctggaag

SEQ ID NO: 168 - RNA, 13 nt, synthetic construct
  misc_feature 1..13: note = Synthetic sequence
  misc_feature 1..13: note = U can be replaced by T. Any base can be replaced with a modified base.
  source 1..13: mol_type = other RNA
caggcagctggaa

SEQ ID NO: 169 - RNA, 13 nt, synthetic construct
  misc_feature 1..13: note = Synthetic sequence
  misc_feature 1..13: note = U can be replaced by T. Any base can be replaced with a modified base.
  source 1..13: mol_type = other RNA
ccaggcagctgga

SEQ ID NO: 170 - RNA, 13 nt, synthetic construct
  misc_feature 1..13: note = Synthetic sequence
  misc_feature 1..13: note = U can be replaced by T. Any base can be replaced with a modified base.
  source 1..13: mol_type = other RNA
cccaggcagctgg

SEQ ID NO: 171 - RNA, 13 nt, synthetic construct
  misc_feature 1..13: note = Synthetic sequence
  misc_feature 1..13: note = U can be replaced by T. Any base can be replaced with a modified base.
  source 1..13: mol_type = other RNA
acccaggcagctg

SEQ ID NO: 172 - RNA, 13 nt, synthetic construct
  misc_feature 1..13: note = Synthetic sequence
  misc_feature 1..13: note = U can be replaced by T. Any base can be replaced with a modified base.
  source 1..13: mol_type = other RNA
aacccaggcagct

SEQ ID NO: 173 - RNA, 13 nt, synthetic construct
  misc_feature 1..13: note = Synthetic sequence
  misc_feature 1..13: note = U can be replaced by T. Any base can be replaced with a modified base.
  source 1..13: mol_type = other RNA
aaacccaggcagc

SEQ ID NO: 174 - RNA, 13 nt, synthetic construct
  misc_feature 1..13: note = Synthetic sequence
  misc_feature 1..13: note = U can be replaced by T. Any base can be replaced with a modified base.
  source 1..13: mol_type = other RNA
gaaacccaggcag

SEQ ID NO: 175 - RNA, 13 nt, synthetic construct
  misc_feature 1..13: note = Synthetic sequence
  misc_feature 1..13: note = U can be replaced by T. Any base can be replaced with a modified base.
  source 1..13: mol_type = other RNA
ggaaacccaggca

SEQ ID NO: 176 - RNA, 13 nt, synthetic construct
  misc_feature 1..13: note = Synthetic sequence
  misc_feature 1..13: note = U can be replaced by T. Any base can be replaced with a modified base.
  source 1..13: mol_type = other RNA
aggaaacccaggc

SEQ ID NO: 177 - RNA, 13 nt, synthetic construct
  misc_feature 1..13: note = Synthetic sequence
  misc_feature 1..13: note = U can be replaced by T. Any base can be replaced with a modified base.
  source 1..13: mol_type = other RNA
caggaaacccagg

SEQ ID NO: 178 - RNA, 13 nt, synthetic construct
  misc_feature 1..13: note = Synthetic sequence
  misc_feature 1..13: note = U can be replaced by T. Any base can be replaced with a modified base.
  source 1..13: mol_type = other RNA
ccaggaaacccag

SEQ ID NO: 179 - RNA, 13 nt, synthetic construct
  misc_feature 1..13: note = Synthetic sequence
  misc_feature 1..13: note = U can be replaced by T. Any base can be replaced with a modified base.
  source 1..13: mol_type = other RNA
tccaggaaaccca

SEQ ID NO: 180 - RNA, 13 nt, synthetic construct
  misc_feature 1..13: note = Synthetic sequence
  misc_feature 1..13: note = U can be replaced by T. Any base can be replaced with a modified base.
  source 1..13: mol_type = other RNA
ttccaggaaaccc

SEQ ID NO: 181 - RNA, 13 nt, synthetic construct
  misc_feature 1..13: note = Synthetic sequence
  misc_feature 1..13: note = U can be replaced by T. Any base can be replaced with a modified base.
  source 1..13: mol_type = other RNA
tttccaggaaacc

SEQ ID NO: 182 - RNA, 13 nt, synthetic construct
  misc_feature 1..13: note = Synthetic sequence
  misc_feature 1..13: note = U can be replaced by T. Any base can be replaced with a modified base.
  source 1..13: mol_type = other RNA
ctttccaggaaac

SEQ ID NO: 183 - RNA, 13 nt, synthetic construct
  misc_feature 1..13: note = Synthetic sequence
  misc_feature 1..13: note = U can be replaced by T. Any base can be replaced with a modified base.
  source 1..13: mol_type = other RNA
tctttccaggaaa

SEQ ID NO: 184 - RNA, 13 nt, synthetic construct
  misc_feature 1..13: note = Synthetic sequence
  misc_feature 1..13: note = U can be replaced by T. Any base can be replaced with a modified base.
  source 1..13: mol_type = other RNA
ttctttccaggaa

SEQ ID NO: 185 - RNA, 13 nt, synthetic construct
  misc_feature 1..13: note = Synthetic sequence
  misc_feature 1..13: note = U can be replaced by T. Any base can be replaced with a modified base.
  source 1..13: mol_type = other RNA
gttctttccagga

SEQ ID NO: 186 - RNA, 13 nt, synthetic construct
  misc_feature 1..13: note = Synthetic sequence
  misc_feature 1..13: note = U can be replaced by T. Any base can be replaced with a modified base.
  source 1..13: mol_type = other RNA
agttctttccagg

SEQ ID NO: 187 - RNA, 13 nt, synthetic construct
  misc_feature 1..13: note = Synthetic sequence
  misc_feature 1..13: note = U can be replaced by T. Any base can be replaced with a modified base.
  source 1..13: mol_type = other RNA
gagttctttccag

SEQ ID NO: 188 - RNA, 13 nt, synthetic construct
  misc_feature 1..13: note = Synthetic sequence
  misc_feature 1..13: note = U can be replaced by T. Any base can be replaced with a modified base.
  source 1..13: mol_type = other RNA
agagttctttcca

SEQ ID NO: 189 - RNA, 13 nt, synthetic construct
  misc_feature 1..13: note = Synthetic sequence
  misc_feature 1..13: note = U can be replaced by T. Any base can be replaced with a modified base.
  source 1..13: mol_type = other RNA
aagagttctttcc

SEQ ID NO: 190 - RNA, 13 nt, synthetic construct
  misc_feature 1..13: note = Synthetic sequence
  misc_feature 1..13: note = U can be replaced by T. Any base can be replaced with a modified base.
  source 1..13: mol_type = other RNA
taagagttctttc

SEQ ID NO: 191 - RNA, 13 nt, synthetic construct
  misc_feature 1..13: note = Synthetic sequence
  misc_feature 1..13: note = U can be replaced by T. Any base can be replaced with a modified base.
  source 1..13: mol_type = other RNA
ataagagttcttt

SEQ ID NO: 192 - RNA, 13 nt, synthetic construct
  misc_feature 1..13: note = Synthetic sequence
  misc_feature 1..13: note = U can be replaced by T. Any base can be replaced with a modified base.
  source 1..13: mol_type = other RNA
gataagagttctt

SEQ ID NO: 193 - RNA, 13 nt, synthetic construct
  misc_feature 1..13: note = Synthetic sequence
  misc_feature 1..13: note = U can be replaced by T. Any base can be replaced with a modified base.
  source 1..13: mol_type = other RNA
ggataagagttct

SEQ ID NO: 194 - RNA, 13 nt, synthetic construct
  misc_feature 1..13: note = Synthetic sequence
  misc_feature 1..13: note = U can be replaced by T. Any base can be replaced with a modified base.
  source 1..13: mol_type = other RNA
gggataagagttc

SEQ ID NO: 195 - RNA, 13 nt, synthetic construct
  misc_feature 1..13: note = Synthetic sequence
  misc_feature 1..13: note = U can be replaced by T. Any base can be replaced with a modified base.
  source 1..13: mol_type = other RNA
ggggataagagtt

SEQ ID NO: 196 - RNA, 13 nt, synthetic construct
  misc_feature 1..13: note = Synthetic sequence
  misc_feature 1..13: note = U can be replaced by T. Any base can be replaced with a modified base.
  source 1..13: mol_type = other RNA
tggggataagagt

SEQ ID NO: 197 - RNA, 13 nt, synthetic construct
  misc_feature 1..13: note = Synthetic sequence
  misc_feature 1..13: note = U can be replaced by T. Any base can be replaced with a modified base.
  source 1..13: mol_type = other RNA
ctggggataagag

SEQ ID NO: 198 - RNA, 13 nt, synthetic construct
  misc_feature 1..13: note = Synthetic sequence
  misc_feature 1..13: note = U can be replaced by T. Any base can be replaced with a modified base.
  source 1..13: mol_type = other RNA
cctggggataaga

SEQ ID NO: 199 - RNA, 13 nt, synthetic construct
  misc_feature 1..13: note = Synthetic sequence
  misc_feature 1..13: note = U can be replaced by T. Any base can be replaced with a modified base.
  source 1..13: mol_type = other RNA
tcctggggataag

SEQ ID NO: 200 - RNA, 13 nt, synthetic construct
  misc_feature 1..13: note = Synthetic sequence
  misc_feature 1..13: note = U can be replaced by T. Any base can be replaced with a modified base.
  source 1..13: mol_type = other RNA
ttcctggggataa

SEQ ID NO: 201 - RNA, 13 nt, synthetic construct
  misc_feature 1..13: note = Synthetic sequence
  misc_feature 1..13: note = U can be replaced by T. Any base can be replaced with a modified base.
  source 1..13: mol_type = other RNA
gttcctggggata

SEQ ID NO: 202 - RNA, 13 nt, synthetic construct
  misc_feature 1..13: note = Synthetic sequence
  misc_feature 1..13: note = U can be replaced by T. Any base can be replaced with a modified base.
  source 1..13: mol_type = other RNA
agttcctggggat

SEQ ID NO: 203 - RNA, 13 nt, synthetic construct
  misc_feature 1..13: note = Synthetic sequence
  misc_feature 1..13: note = U can be replaced by T. Any base can be replaced with a modified base.
  source 1..13: mol_type = other RNA
tagttcctgggga

SEQ ID NO: 204 - RNA, 13 nt, synthetic construct
  misc_feature 1..13: note = Synthetic sequence
  misc_feature 1..13: note = U can be replaced by T. Any base can be replaced with a modified base.
  source 1..13: mol_type = other RNA
ctagttcctgggg

SEQ ID NO: 205 - RNA, 13 nt, synthetic construct
  misc_feature 1..13: note = Synthetic sequence
  misc_feature 1..13: note = U can be replaced by T. Any base can be replaced with a modified base.
  source 1..13: mol_type = other RNA
actagttcctggg

SEQ ID NO: 206 - RNA, 13 nt, synthetic construct
  misc_feature 1..13: note = Synthetic sequence
  misc_feature 1..13: note = U can be replaced by T. Any base can be replaced with a modified base.
  source 1..13: mol_type = other RNA
aactagttcctgg

SEQ ID NO: 207 - RNA, 13 nt, synthetic construct
  misc_feature 1..13: note = Synthetic sequence
  misc_feature 1..13: note = U can be replaced by T. Any base can be replaced with a modified base.
  source 1..13: mol_type = other RNA
aaactagttcctg

SEQ ID NO: 208 - RNA, 13 nt, synthetic construct
  misc_feature 1..13: note = Synthetic sequence
  misc_feature 1..13: note = U can be replaced by T. Any base can be replaced with a modified base.
  source 1..13: mol_type = other RNA
caaactagttcct

SEQ ID NO: 209 - RNA, 13 nt, synthetic construct
  misc_feature 1..13: note = Synthetic sequence
  misc_feature 1..13: note = U can be replaced by T. Any base can be replaced with a modified base.
  source 1..13: mol_type = other RNA
acaaactagttcc

SEQ ID NO: 210 - RNA, 13 nt, synthetic construct
  misc_feature 1..13: note = Synthetic sequence
  misc_feature 1..13: note = U can be replaced by T. Any base can be replaced with a modified base.
  source 1..13: mol_type = other RNA
aacaaactagttc

SEQ ID NO: 211 - RNA, 13 nt, synthetic construct
  misc_feature 1..13: note = Synthetic sequence
  misc_feature 1..13: note = U can be replaced by T. Any base can be replaced with a modified base.
  source 1..13: mol_type = other RNA
caacaaactagtt

SEQ ID NO: 212 - RNA, 13 nt, synthetic construct
  misc_feature 1..13: note = Synthetic sequence
  misc_feature 1..13: note = U can be replaced by T. Any base can be replaced with a modified base.
  source 1..13: mol_type = other RNA
tcaacaaactagt

SEQ ID NO: 213 - RNA, 13 nt, synthetic construct
  misc_feature 1..13: note = Synthetic sequence
  misc_feature 1..13: note = U can be replaced by T. Any base can be replaced with a modified base.
  source 1..13: mol_type = other RNA
ttcaacaaactag

SEQ ID NO: 214 - RNA, 13 nt, synthetic construct
  misc_feature 1..13: note = Synthetic sequence
  misc_feature 1..13: note = U can be replaced by T. Any base can be replaced with a modified base.
  source 1..13: mol_type = other RNA
attcaacaaacta

SEQ ID NO: 215 - RNA, 13 nt, synthetic construct
  misc_feature 1..13: note = Synthetic sequence
  misc_feature 1..13: note = U can be replaced by T. Any base can be replaced with a modified base.
  source 1..13: mol_type = other RNA
tattcaacaaact

SEQ ID NO: 216 - RNA, 13 nt, synthetic construct
  misc_feature 1..13: note = Synthetic sequence
  misc_feature 1..13: note = U can be replaced by T. Any base can be replaced with a modified base.
  source 1..13: mol_type = other RNA
ttattcaacaaac

SEQ ID NO: 217 - RNA, 13 nt, synthetic construct
  misc_feature 1..13: note = Synthetic sequence
  misc_feature 1..13: note = U can be replaced by T. Any base can be replaced with a modified base.
  source 1..13: mol_type = other RNA
tttattcaacaaa

SEQ ID NO: 218 - RNA, 13 nt, synthetic construct
  misc_feature 1..13: note = Synthetic sequence
  misc_feature 1..13: note = U can be replaced by T. Any base can be replaced with a modified base.
  source 1..13: mol_type = other RNA
atttattcaacaa

SEQ ID NO: 219 - RNA, 13 nt, synthetic construct
  misc_feature 1..13: note = Synthetic sequence
  misc_feature 1..13: note = U can be replaced by T. Any base can be replaced with a modified base.
  source 1..13: mol_type = other RNA
catttattcaaca

SEQ ID NO: 220 - RNA, 13 nt, synthetic construct
  misc_feature 1..13: note = Synthetic sequence
  misc_feature 1..13: note = U can be replaced by T. Any base can be replaced with a modified base.
  source 1..13: mol_type = other RNA
gcatttattcaac

SEQ ID NO: 221 - RNA, 13 nt, synthetic construct
  misc_feature 1..13: note = Synthetic sequence
  misc_feature 1..13: note = U can be replaced by T. Any base can be replaced with a modified base.
  source 1..13: mol_type = other RNA
agcatttattcaa

SEQ ID NO: 222 - RNA, 13 nt, synthetic construct
  misc_feature 1..13: note = Synthetic sequence
  misc_feature 1..13: note = U can be replaced by T. Any base can be replaced with a modified base.
  source 1..13: mol_type = other RNA
cagcatttattca

SEQ ID NO: 223 - RNA, 13 nt, synthetic construct
  misc_feature 1..13: note = Synthetic sequence
  misc_feature 1..13: note = U can be replaced by T. Any base can be replaced with a modified base.
  source 1..13: mol_type = other RNA
ccagcatttattc

SEQ ID NO: 224 - RNA, 13 nt, synthetic construct
  misc_feature 1..13: note = Synthetic sequence
  misc_feature 1..13: note = U can be replaced by T. Any base can be replaced with a modified base.
  source 1..13: mol_type = other RNA
accagcatttatt

SEQ ID NO: 225 - RNA, 13 nt, synthetic construct
  misc_feature 1..13: note = Synthetic sequence
  misc_feature 1..13: note = U can be replaced by T. Any base can be replaced with a modified base.
  source 1..13: mol_type = other RNA
caccagcatttat

SEQ ID NO: 226 - RNA, 13 nt, synthetic construct
  misc_feature 1..13: note = Synthetic sequence
  misc_feature 1..13: note = U can be replaced by T. Any base can be replaced with a modified base.
  source 1..13: mol_type = other RNA
tcaccagcattta

SEQ ID NO: 227 - RNA, 13 nt, synthetic construct
  misc_feature 1..13: note = Synthetic sequence
  misc_feature 1..13: note = U can be replaced by T. Any base can be replaced with a modified base.
  source 1..13: mol_type = other RNA
ttcaccagcattt

SEQ ID NO: 228 - RNA, 13 nt, synthetic construct
  misc_feature 1..13: note = Synthetic sequence
  misc_feature 1..13: note = U can be replaced by T. Any base can be replaced with a modified base.
  source 1..13: mol_type = other RNA
attcaccagcatt

SEQ ID NO: 229 - RNA, 13 nt, synthetic construct
  misc_feature 1..13: note = Synthetic sequence
  misc_feature 1..13: note = U can be replaced by T. Any base can be replaced with a modified base.
  source 1..13: mol_type = other RNA
cattcaccagcat

SEQ ID NO: 230 - RNA, 13 nt, synthetic construct
  misc_feature 1..13: note = Synthetic sequence
  misc_feature 1..13: note = U can be replaced by T. Any base can be replaced with a modified base.
  source 1..13: mol_type = other RNA
tcattcaccagca

SEQ ID NO: 231 - RNA, 13 nt, synthetic construct
  misc_feature 1..13: note = Synthetic sequence
  misc_feature 1..13: note = U can be replaced by T. Any base can be replaced with a modified base.
  source 1..13: mol_type = other RNA
ttcattcaccagc

SEQ ID NO: 232 - RNA, 13 nt, synthetic construct
  misc_feature 1..13: note = Synthetic sequence
  misc_feature 1..13: note = U can be replaced by T. Any base can be replaced with a modified base.
  source 1..13: mol_type = other RNA
attcattcaccag

SEQ ID NO: 233 - RNA, 13 nt, synthetic construct
  misc_feature 1..13: note = Synthetic sequence
  misc_feature 1..13: note = U can be replaced by T. Any base can be replaced with a modified base.
  source 1..13: mol_type = other RNA
cattcattcacca

SEQ ID NO: 234 - RNA, 13 nt, synthetic construct
  misc_feature 1..13: note = Synthetic sequence
  misc_feature 1..13: note = U can be replaced by T. Any base can be replaced with a modified base.
  source 1..13: mol_type = other RNA
tcattcattcacc

SEQ ID NO: 235 - RNA, 13 nt, synthetic construct
  misc_feature 1..13: note = Synthetic sequence
  misc_feature 1..13: note = U can be replaced by T. Any base can be replaced with a modified base.
  source 1..13: mol_type = other RNA
ttcattcattcac

SEQ ID NO: 236 - RNA, 13 nt, synthetic construct
  misc_feature 1..13: note = Synthetic sequence
  misc_feature 1..13: note = U can be replaced by T. Any base can be replaced with a modified base.
  source 1..13: mol_type = other RNA
attcattcattca

SEQ ID NO: 237 - RNA, 13 nt, synthetic construct
  misc_feature 1..13: note = Synthetic sequence
  misc_feature 1..13: note = U can be replaced by T. Any base can be replaced with a modified base.
  source 1..13: mol_type = other RNA
cattcattcattc

SEQ ID NO: 238 - RNA, 13 nt, synthetic construct
  misc_feature 1..13: note = Synthetic sequence
  misc_feature 1..13: note = U can be replaced by T. Any base can be replaced with a modified base.
  source 1..13: mol_type = other RNA
tcattcattcatt

SEQ ID NO: 239 - RNA, 13 nt, synthetic construct
  misc_feature 1..13: note = Synthetic sequence
  misc_feature 1..13: note = U can be replaced by T. Any base can be replaced with a modified base.
  source 1..13: mol_type = other RNA
atcattcattcat

SEQ ID NO: 240 - RNA, 13 nt, synthetic construct
  misc_feature 1..13: note = Synthetic sequence
  misc_feature 1..13: note = U can be replaced by T. Any base can be replaced with a modified base.
  source 1..13: mol_type = other RNA
aatcattcattca

SEQ ID NO: 241 - RNA, 13 nt, synthetic construct
  misc_feature 1..13: note = Synthetic sequence
  misc_feature 1..13: note = U can be replaced by T. Any base can be replaced with a modified base.
  source 1..13: mol_type = other RNA
caatcattcattc

SEQ ID NO: 242 - RNA, 13 nt, synthetic construct
  misc_feature 1..13: note = Synthetic sequence
  misc_feature 1..13: note = U can be replaced by T. Any base can be replaced with a modified base.
  source 1..13: mol_type = other RNA
tcaatcattcatt

SEQ ID NO: 243 - RNA, 13 nt, synthetic construct
  misc_feature 1..13: note = Synthetic sequence
  misc_feature 1..13: note = U can be replaced by T. Any base can be replaced with a modified base.
  source 1..13: mol_type = other RNA
ttcaatcattcat

SEQ ID NO: 244 - RNA, 13 nt, synthetic construct
  misc_feature 1..13: note = Synthetic sequence
  misc_feature 1..13: note = U can be replaced by T. Any base can be replaced with a modified base.
  source 1..13: mol_type = other RNA
gttcaatcattca

SEQ ID NO: 245 - RNA, 13 nt, synthetic construct
  misc_feature 1..13: note = Synthetic sequence
  misc_feature 1..13: note = U can be replaced by T. Any base can be replaced with a modified base.
  source 1..13: mol_type = other RNA
tgttcaatcattc

SEQ ID NO: 246 - RNA, 13 nt, synthetic construct
  misc_feature 1..13: note = Synthetic sequence
  misc_feature 1..13: note = U can be replaced by T. Any base can be replaced with a modified base.
  source 1..13: mol_type = other RNA
ctgttcaatcatt

SEQ ID NO: 247 - RNA, 13 nt, synthetic construct
  misc_feature 1..13: note = Synthetic sequence
  misc_feature 1..13: note = U can be replaced by T. Any base can be replaced with a modified base.
  source 1..13: mol_type = other RNA
tctgttcaatcat

SEQ ID NO: 248 - RNA, 13 nt, synthetic construct
  misc_feature 1..13: note = Synthetic sequence
  misc_feature 1..13: note = U can be replaced by T. Any base can be replaced with a modified base.
  source 1..13: mol_type = other RNA
atctgttcaatca

SEQ ID NO: 249 - RNA, 13 nt, synthetic construct
  misc_feature 1..13: note = Synthetic sequence
  misc_feature 1..13: note = U can be replaced by T. Any base can be replaced with a modified base.
  source 1..13: mol_type = other RNA
catctgttcaatc

SEQ ID NO: 250 - RNA, 13 nt, synthetic construct
  misc_feature 1..13: note = Synthetic sequence
  misc_feature 1..13: note = U can be replaced by T. Any base can be replaced with a modified base.
  source 1..13: mol_type = other RNA
tcatctgttcaat

SEQ ID NO: 251 - RNA, 13 nt, synthetic construct
  misc_feature 1..13: note = Synthetic sequence
  misc_feature 1..13: note = U can be replaced by T. Any base can be replaced with a modified base.
  source 1..13: mol_type = other RNA
ttcatctgttcaa

SEQ ID NO: 252 - RNA, 13 nt, synthetic construct
  misc_feature 1..13: note = Synthetic sequence
  misc_feature 1..13: note = U can be replaced by T. Any base can be replaced with a modified base.
  source 1..13: mol_type = other RNA
attcatctgttca

SEQ ID NO: 253 - RNA, 13 nt, synthetic construct
  misc_feature 1..13: note = Synthetic sequence
  misc_feature 1..13: note = U can be replaced by T. Any base can be replaced with a modified base.
  source 1..13: mol_type = other RNA
cattcatctgttc

SEQ ID NO: 254 - RNA, 13 nt, synthetic construct
  misc_feature 1..13: note = Synthetic sequence
  misc_feature 1..13: note = U can be replaced by T. Any base can be replaced with a modified base.
  source 1..13: mol_type = other RNA
tcattcatctgtt

SEQ ID NO: 255 - RNA, 13 nt, synthetic construct
  misc_feature 1..13: note = Synthetic sequence
  misc_feature 1..13: note = U can be replaced by T. Any base can be replaced with a modified base.
  source 1..13: mol_type = other RNA
ctcattcatctgt

SEQ ID NO: 256 - RNA, 13 nt, synthetic construct
  misc_feature 1..13: note = Synthetic sequence
  misc_feature 1..13: note = U can be replaced by T. Any base can be replaced with a modified base.
  source 1..13: mol_type = other RNA
actcattcatctg

SEQ ID NO: 257 - RNA, 13 nt, synthetic construct
  misc_feature 1..13: note = Synthetic sequence
  misc_feature 1..13: note = U can be replaced by T. Any base can be replaced with a modified base.
  source 1..13: mol_type = other RNA
cactcattcatct

SEQ ID NO: 258 - RNA, 13 nt, synthetic construct
  misc_feature 1..13: note = Synthetic sequence
  misc_feature 1..13: note = U can be replaced by T. Any base can be replaced with a modified base.
  source 1..13: mol_type = other RNA
tcactcattcatc

SEQ ID NO: 259 - RNA, 13 nt, synthetic construct
  misc_feature 1..13: note = Synthetic sequence
  misc_feature 1..13: note = U can be replaced by T. Any base can be replaced with a modified base.
  source 1..13: mol_type = other RNA
atcactcattcat

SEQ ID NO: 260 - RNA, 13 nt, synthetic construct
  misc_feature 1..13: note = Synthetic sequence
  misc_feature 1..13: note = U can be replaced by T. Any base can be replaced with a modified base.
  source 1..13: mol_type = other RNA
catcactcattca

SEQ ID NO: 261 - RNA, 13 nt, synthetic construct
  misc_feature 1..13: note = Synthetic sequence
  misc_feature 1..13: note = U can be replaced by T. Any base can be replaced with a modified base.
  source 1..13: mol_type = other RNA
tcatcactcattc

SEQ ID NO: 262 - RNA, 13 nt, synthetic construct
  misc_feature 1..13: note = Synthetic sequence
  misc_feature 1..13: note = U can be replaced by T. Any base can be replaced with a modified base.
  source 1..13: mol_type = other RNA
ctcatcactcatt

SEQ ID NO: 263 - RNA, 13 nt, synthetic construct
  misc_feature 1..13: note = Synthetic sequence
  misc_feature 1..13: note = U can be replaced by T. Any base can be replaced with a modified base.
  source 1..13: mol_type = other RNA
actcatcactcat

SEQ ID NO: 264 - RNA, 13 nt, synthetic construct
  misc_feature 1..13: note = Synthetic sequence
  misc_feature 1..13: note = U can be replaced by T. Any base can be replaced with a modified base.
  source 1..13: mol_type = other RNA
tactcatcactca

SEQ ID NO: 265 - RNA, 13 nt, synthetic construct
  misc_feature 1..13: note = Synthetic sequence
  misc_feature 1..13: note = U can be replaced by T. Any base can be replaced with a modified base.
  source 1..13: mol_type = other RNA
ctactcatcactc

SEQ ID NO: 266 - RNA, 13 nt, synthetic construct
  misc_feature 1..13: note = Synthetic sequence
  misc_feature 1..13: note = U can be replaced by T. Any base can be replaced with a modified base.
  source 1..13: mol_type = other RNA
tctactcatcact

SEQ ID NO: 267 - RNA, 13 nt, synthetic construct
  misc_feature 1..13: note = Synthetic sequence
  misc_feature 1..13: note = U can be replaced by T. Any base can be replaced with a modified base.
  source 1..13: mol_type = other RNA
atctactcatcac

SEQ ID NO: 268 - RNA, 13 nt, synthetic construct
  misc_feature 1..13: note = Synthetic sequence
  misc_feature 1..13: note = U can be replaced by T. Any base can be replaced with a modified base.
  source 1..13: mol_type = other RNA
tatctactcatca

SEQ ID NO: 269 - RNA, 13 nt, synthetic construct
  misc_feature 1..13: note = Synthetic sequence
  misc_feature 1..13: note = U can be replaced by T. Any base can be replaced with a modified base.
  source 1..13: mol_type = other RNA
ttatctactcatc

SEQ ID NO: 270 - RNA, 13 nt, synthetic construct
  misc_feature 1..13: note = Synthetic sequence
  misc_feature 1..13: note = U can be replaced by T. Any base can be replaced with a modified base.
  source 1..13: mol_type = other RNA
tttatctactcat

SEQ ID NO: 271 - RNA, 13 nt, synthetic construct
  misc_feature 1..13: note = Synthetic sequence
  misc_feature 1..13: note = U can be replaced by T. Any base can be replaced with a modified base.
  source 1..13: mol_type = other RNA
ttttatctactca

SEQ ID NO: 272 - RNA, 13 nt, synthetic construct
  misc_feature 1..13: note = Synthetic sequence
  misc_feature 1..13: note = U can be replaced by T. Any base can be replaced with a modified base.
  source 1..13: mol_type = other RNA
cttttatctactc

SEQ ID NO: 273 - RNA, 13 nt, synthetic construct
  misc_feature 1..13: note = Synthetic sequence
  misc_feature 1..13: note = U can be replaced by T. Any base can be replaced with a modified base.
  source 1..13: mol_type = other RNA
ccttttatctact

SEQ ID NO: 274 - RNA, 13 nt, synthetic construct
  misc_feature 1..13: note = Synthetic sequence
  misc_feature 1..13: note = U can be replaced by T. Any base can be replaced with a modified base.
  source 1..13: mol_type = other RNA
gcttttatctact

SEQ ID NO: 275 - RNA, 13 nt, synthetic construct
  misc_feature 1..13: note = Synthetic sequence
  misc_feature 1..13: note = U can be replaced by T. Any base can be replaced with a modified base.
  source 1..13: mol_type = other RNA
tccttttatctac

SEQ ID NO: 276 - RNA, 13 nt, synthetic construct
  misc_feature 1..13: note = Synthetic sequence
  misc_feature 1..13: note = U can be replaced by T. Any base can be replaced with a modified base.
  source 1..13: mol_type = other RNA
tgcttttatctac

SEQ ID NO: 277 - RNA, 13 nt, synthetic construct
  misc_feature 1..13: note = Synthetic sequence
  misc_feature 1..13: note = U can be replaced by T. Any base can be replaced with a modified base.
  source 1..13: mol_type = other RNA
atccttttatcta

SEQ ID NO: 278 - RNA, 13 nt, synthetic construct
  misc_feature 1..13: note = Synthetic sequence
  misc_feature 1..13: note = U can be replaced by T. Any base can be replaced with a modified base.
  source 1..13: mol_type = other RNA
atgcttttatcta

SEQ ID NO: 279 - RNA, 13 nt, synthetic construct
  misc_feature 1..13: note = Synthetic sequence
  misc_feature 1..13: note = U can be replaced by T. Any base can be replaced with a modified base.
  source 1..13: mol_type = other RNA
catccttttatct

SEQ ID NO: 280 - RNA, 13 nt, synthetic construct
  misc_feature 1..13: note = Synthetic sequence
  misc_feature 1..13: note = U can be replaced by T. Any base can be replaced with a modified base.
  source 1..13: mol_type = other RNA
catgcttttatct

SEQ ID NO: 281 - RNA, 13 nt, synthetic construct
  misc_feature 1..13: note = Synthetic sequence
  source 1..13: mol_type = other RNA
ccatccttttatc

SEQ ID NO: 282 - RNA, 13 nt, synthetic construct
  misc_feature 1..13: note = Synthetic sequence
  misc_feature 1..13: note = U can be replaced by T. Any base can be replaced with a modified base.
  source 1..13: mol_type = other RNA
ccatgcttttatc

SEQ ID NO: 283 - RNA, 13 nt, synthetic construct
  misc_feature 1..13: note = Synthetic sequence
  misc_feature 1..13: note = U can be replaced by T. Any base can be replaced with a modified base.
  source 1..13: mol_type = other RNA
tccatccttttat

SEQ ID NO: 284 - RNA, 13 nt, synthetic construct
  misc_feature 1..13: note = Synthetic sequence
  misc_feature 1..13: note = U can be replaced by T. Any base can be replaced with a modified base.
  source 1..13: mol_type = other RNA
tccatgcttttat

SEQ ID NO: 285 - RNA, 13 nt, synthetic construct
  misc_feature 1..13: note = Synthetic sequence
  misc_feature 1..13: note = U can be replaced by T. Any base can be replaced with a modified base.
  source 1..13: mol_type = other RNA
atccatcctttta

SEQ ID NO: 286 - RNA, 13 nt, synthetic construct
  misc_feature 1..13: note = Synthetic sequence
  misc_feature 1..13: note = U can be replaced by T. Any base can be replaced with a modified base.
  source 1..13: mol_type = other RNA
atccatgctttta

SEQ ID NO: 287 - RNA, 13 nt, synthetic construct
  misc_feature 1..13: note = Synthetic sequence
  misc_feature 1..13: note = U can be replaced by T. Any base can be replaced with a modified base.
  source 1..13: mol_type = other RNA
catccatcctttt

SEQ ID NO: 288 - RNA, 13 nt, synthetic construct
  misc_feature 1..13: note = Synthetic sequence
  misc_feature 1..13: note = U can be replaced by T. Any base can be replaced with a modified base.
  source 1..13: mol_type = other RNA
catccatgctttt

SEQ ID NO: 289 - RNA, 13 nt, synthetic construct
  misc_feature 1..13: note = Synthetic sequence
  misc_feature 1..13: note = U can be replaced by T. Any base can be replaced with a modified base.
  source 1..13: mol_type = other RNA
ccatccatccttt

SEQ ID NO: 290 - RNA, 13 nt, synthetic construct
  misc_feature 1..13: note = Synthetic sequence
  misc_feature 1..13: note = U can be replaced by T. Any base can be replaced with a modified base.
  source 1..13: mol_type = other RNA
ccatccatgcttt

SEQ ID NO: 291 - RNA, 13 nt, synthetic construct
  misc_feature 1..13: note = Synthetic sequence
  misc_feature 1..13: note = U can be replaced by T. Any base can be replaced with a modified base.
  source 1..13: mol_type = other RNA
tccatccatcctt

SEQ ID NO: 292 - RNA, 13 nt, synthetic construct
  misc_feature 1..13: note = Synthetic sequence
  misc_feature 1..13: note = U can be replaced by T. Any base can be replaced with a modified base.
  source 1..13: mol_type = other RNA
tccatccatgctt

SEQ ID NO: 293 - RNA, 13 nt, synthetic construct
  misc_feature 1..13: note = Synthetic sequence
  misc_feature 1..13: note = U can be replaced by T. Any base can be replaced with a modified base.
  source 1..13: mol_type = other RNA
ctccatccatcct

SEQ ID NO: 294 - RNA, 13 nt, synthetic construct
  misc_feature 1..13: note = Synthetic sequence
  misc_feature 1..13: note = U can be replaced by T. Any base can be replaced with a modified base.
  source 1..13: mol_type = other RNA
ctccatccatgct

SEQ ID NO: 295 - RNA, 13 nt, synthetic construct
  misc_feature 1..13: note = Synthetic sequence
  misc_feature 1..13: note = U can be replaced by T. Any base can be replaced with a modified base.
  source 1..13: mol_type = other RNA
tctccatccatcc

SEQ ID NO: 296 - RNA, 13 nt, synthetic construct
  misc_feature 1..13: note = Synthetic sequence
  misc_feature 1..13: note = U can be replaced by T. Any base can be replaced with a modified base.
  source 1..13: mol_type = other RNA
tctccatccatgc

SEQ ID NO: 297 - RNA, 13 nt, synthetic construct
  misc_feature 1..13: note = Synthetic sequence
  misc_feature 1..13: note = U can be replaced by T. Any base can be replaced with a modified base.
  source 1..13: mol_type = other RNA
ctctccatccatc

SEQ ID NO: 298 - RNA, 13 nt, synthetic construct
  misc_feature 1..13: note = Synthetic sequence
  misc_feature 1..13: note = U can be replaced by T. Any base can be replaced with a modified base.
  source 1..13: mol_type = other RNA
ctctccatccatg

SEQ ID NO: 299 - RNA, 13 nt, synthetic construct
  misc_feature 1..13: note = Synthetic sequence
  misc_feature 1..13: note = U can be replaced by T. Any base can be replaced with a modified base.
  source 1..13: mol_type = other RNA
tctctccatccat

SEQ ID NO: 300 - RNA, 13 nt, synthetic construct
  misc_feature 1..13: note = Synthetic sequence
  misc_feature 1..13: note = U can be replaced by T. Any base can be replaced with a modified base.
  source 1..13: mol_type = other RNA
atctctccatcca

SEQ ID NO: 301 - RNA, 13 nt, synthetic construct
  misc_feature 1..13: note = Synthetic sequence
  misc_feature 1..13: note = U can be replaced by T. Any base can be replaced with a modified base.
  source 1..13: mol_type = other RNA
catctctccatcc

SEQ ID NO: 302 - RNA, 13 nt, synthetic construct
  misc_feature 1..13: note = Synthetic sequence
  misc_feature 1..13: note = U can be replaced by T. Any base can be replaced with a modified base.
  source 1..13: mol_type = other RNA
ccatctctccatc

SEQ ID NO: 303 - RNA, 13 nt, synthetic construct
  misc_feature 1..13: note = Synthetic sequence
  misc_feature 1..13: note = U can be replaced by T. Any base can be replaced with a modified base.
  source 1..13: mol_type = other RNA
cccatctctccat

SEQ ID NO: 304 - RNA, 13 nt, synthetic construct
  misc_feature 1..13: note = Synthetic sequence
  misc_feature 1..13: note = U can be replaced by T. Any base can be replaced with a modified base.
  source 1..13: mol_type = other RNA
acccatctctcca

SEQ ID NO: 305 - RNA, 13 nt, synthetic construct
  misc_feature 1..13: note = Synthetic sequence
  misc_feature 1..13: note = U can be replaced by T. Any base can be replaced with a modified base.
  source 1..13: mol_type = other RNA
cacccatctctcc

SEQ ID NO: 306 - RNA, 13 nt, synthetic construct
  misc_feature 1..13: note = Synthetic sequence
  misc_feature 1..13: note = U can be replaced by T. Any base can be replaced with a modified base.
  source 1..13: mol_type = other RNA
tcacccatctctc

SEQ ID NO: 307 - RNA, 13 nt, synthetic construct
  misc_feature 1..13: note = Synthetic sequence
  misc_feature 1..13: note = U can be replaced by T. Any base can be replaced with a modified base.
  source 1..13: mol_type = other RNA
ctcacccatctct

SEQ ID NO: 308 - RNA, 13 nt, synthetic construct
  misc_feature 1..13: note = Synthetic sequence
  misc_feature 1..13: note = U can be replaced by T. Any base can be replaced with a modified base.
  source 1..13: mol_type = other RNA
actcacccatctc

SEQ ID NO: 309 - RNA, 13 nt, synthetic construct
  misc_feature 1..13: note = Synthetic sequence
  misc_feature 1..13: note = U can be replaced by T. Any base can be replaced with a modified base.
  source 1..13: mol_type = other RNA
tactcacccatct

SEQ ID NO: 310 - RNA, 13 nt, synthetic construct
  misc_feature 1..13: note = Synthetic sequence
  misc_feature 1..13: note = U can be replaced by T. Any base can be replaced with a modified base.
  source 1..13: mol_type = other RNA
gtactcacccatc

SEQ ID NO: 311 - RNA, 13 nt, synthetic construct
  misc_feature 1..13: note = Synthetic sequence
  misc_feature 1..13: note = U can be replaced by T. Any base can be replaced with a modified base.
  source 1..13: mol_type = other RNA
tgtactcacccat

SEQ ID NO: 312 - RNA, 13 nt, synthetic construct
  misc_feature 1..13: note = Synthetic sequence
  misc_feature 1..13: note = U can be replaced by T. Any base can be replaced with a modified base.
  source 1..13: mol_type = other RNA
atgtactcaccca

SEQ ID NO: 313 - RNA, 13 nt, synthetic construct
  misc_feature 1..13: note = Synthetic sequence
  misc_feature 1..13: note = U can be replaced by T. Any base can be replaced with a modified base.
  source 1..13: mol_type = other RNA
catgtactcaccc

SEQ ID NO: 314 - RNA, 13 nt, synthetic construct
  misc_feature 1..13: note = Synthetic sequence
  misc_feature 1..13: note = U can be replaced by T. Any base can be replaced with a modified base.
  source 1..13: mol_type = other RNA
ccatgtactcacc

SEQ ID NO: 315 - RNA, 13 nt, synthetic construct
  misc_feature 1..13: note = Synthetic sequence
  misc_feature 1..13: note = U can be replaced by T. Any base can be replaced with a modified base.
  source 1..13: mol_type = other RNA
tccatgtactcac

SEQ ID NO: 316 - RNA, 13 nt, synthetic construct
  misc_feature 1..13: note = Synthetic sequence
  misc_feature 1..13: note = U can be replaced by T. Any base can be replaced with a modified base.
  source 1..13: mol_type = other RNA
atccatgtactca

SEQ ID NO: 317 - RNA, 13 nt, synthetic construct
  misc_feature 1..13: note = Synthetic sequence
  misc_feature 1..13: note = U can be replaced by T. Any base can be replaced with a modified base.
  source 1..13: mol_type = other RNA
catccatgtactc

SEQ ID NO: 318 - RNA, 13 nt, synthetic construct
  misc_feature 1..13: note = Synthetic sequence
  misc_feature 1..13: note = U can be replaced by T. Any base can be replaced with a modified base.
  source 1..13: mol_type = other RNA
ccatccatgtact

SEQ ID NO: 319 - RNA, 13 nt, synthetic construct
  misc_feature 1..13: note = Synthetic sequence
  misc_feature 1..13: note = U can be replaced by T. Any base can be replaced with a modified base.
  source 1..13: mol_type = other RNA
tccatccatgtac

SEQ ID NO: 320 - RNA, 13 nt, synthetic construct
  misc_feature 1..13: note = Synthetic sequence
  misc_feature 1..13: note = U can be replaced by T. Any base can be replaced with a modified base.
  source 1..13: mol_type = other RNA
atccatccatgta

SEQ ID NO: 321 - RNA, 13 nt, synthetic construct
  misc_feature 1..13: note = Synthetic sequence
  misc_feature 1..13: note = U can be replaced by T. Any base can be replaced with a modified base.
  source 1..13: mol_type = other RNA
tatccatccatgt

SEQ ID NO: 322 - RNA, 13 nt, synthetic construct
  misc_feature 1..13: note = Synthetic sequence
  misc_feature 1..13: note = U can be replaced by T. Any base can be replaced with a modified base.
  source 1..13: mol_type = other RNA
ctatccatccatg

SEQ ID NO: 323 - RNA, 13 nt, synthetic construct
  misc_feature 1..13: note = Synthetic sequence
  misc_feature 1..13: note = U can be replaced by T. Any base can be replaced with a modified base.
  source 1..13: mol_type = other RNA
tctatccatccat

SEQ ID NO: 324 - RNA, 13 nt, synthetic construct
  misc_feature 1..13: note = Synthetic sequence
  misc_feature 1..13: note = U can be replaced by T. Any base can be replaced with a modified base.
  source 1..13: mol_type = other RNA
atctatccatcca

SEQ ID NO: 325 - RNA, 13 nt, synthetic construct
  misc_feature 1..13: note = Synthetic sequence
  misc_feature 1..13: note = U can be replaced by T. Any base can be replaced with a modified base.
  source 1..13: mol_type = other RNA
catctatccatcc

SEQ ID NO: 326 - RNA, 13 nt, synthetic construct
  misc_feature 1..13: note = Synthetic sequence
  misc_feature 1..13: note = U can be replaced by T. Any base can be replaced with a modified base.
  source 1..13: mol_type = other RNA
ccatctatccatc

SEQ ID NO: 327 - RNA, 13 nt, synthetic construct
  misc_feature 1..13: note = Synthetic sequence
  misc_feature 1..13: note = U can be replaced by T. Any base can be replaced with a modified base.
  source 1..13: mol_type = other RNA
tccatctatccat

SEQ ID NO: 328 - RNA, 13 nt, synthetic construct
  misc_feature 1..13: note = Synthetic sequence
  misc_feature 1..13: note = U can be replaced by T. Any base can be replaced with a modified base.
  source 1..13: mol_type = other RNA
atccatctatcca

SEQ ID NO: 329 - RNA, 13 nt, synthetic construct
  misc_feature 1..13: note = Synthetic sequence
  misc_feature 1..13: note = U can be replaced by T. Any base can be replaced with a modified base.
  source 1..13: mol_type = other RNA
catccatctatcc

SEQ ID NO: 330 - RNA, 13 nt, synthetic construct
  misc_feature 1..13: note = Synthetic sequence
  misc_feature 1..13: note = U can be replaced by T. Any base can be replaced with a modified base.
  source 1..13: mol_type = other RNA
tcatccatctatc

SEQ ID NO: 331 - RNA, 13 nt, synthetic construct
  misc_feature 1..13: note = Synthetic sequence
  misc_feature 1..13: note = U can be replaced by T. Any base can be replaced with a modified base.
  source 1..13: mol_type = other RNA
ctcatccatctat

SEQ ID NO: 332 - RNA, 13 nt, synthetic construct
  misc_feature 1..13: note = Synthetic sequence
  misc_feature 1..13: note = U can be replaced by T. Any base can be replaced with a modified base.
  source 1..13: mol_type = other RNA
actcatccatcta

SEQ ID NO: 333 - RNA, 13 nt, synthetic construct
  misc_feature 1..13: note = Synthetic sequence
  misc_feature 1..13: note = U can be replaced by T. Any base can be replaced with a modified base.
  source 1..13: mol_type = other RNA
aactcatccatct

SEQ ID NO: 334 - RNA, 13 nt, synthetic construct
  misc_feature 1..13: note = Synthetic sequence
  misc_feature 1..13: note = U can be replaced by T. Any base can be replaced with a modified base.
  source 1..13: mol_type = other RNA
caactcatccatc

SEQ ID NO: 335 - RNA, 13 nt, synthetic construct
  misc_feature 1..13: note = Synthetic sequence
  misc_feature 1..13: note = U can be replaced by T. Any base can be replaced with a modified base.
  source 1..13: mol_type = other RNA
ccaactcatccat

SEQ ID NO: 336 - RNA, 13 nt, synthetic construct
  misc_feature 1..13: note = Synthetic sequence
  misc_feature 1..13: note = U can be replaced by T. Any base can be replaced with a modified base.
  source 1..13: mol_type = other RNA
accaactcatcca

SEQ ID NO: 337 - RNA, 13 nt, synthetic construct
  misc_feature 1..13: note = Synthetic sequence
  misc_feature 1..13: note = U can be replaced by T. Any base can be replaced with a modified base.
  source 1..13: mol_type = other RNA
caccaactcatcc

SEQ ID NO: 338 - RNA, 13 nt, synthetic construct
  misc_feature 1..13: note = Synthetic sequence
  misc_feature 1..13: note = U can be replaced by T. Any base can be replaced with a modified base.
  source 1..13: mol_type = other RNA
ccaccaactcatc

SEQ ID NO: 339 - RNA, 13 nt, synthetic construct
  misc_feature 1..13: note = Synthetic sequence
  misc_feature 1..13: note = U can be replaced by T. Any base can be replaced with a modified base.
  source 1..13: mol_type = other RNA
cccaccaactcat

SEQ ID NO: 340 - RNA, 13 nt, synthetic construct
  misc_feature 1..13: note = Synthetic sequence
  misc_feature 1..13: note = U can be replaced by T. Any base can be replaced with a modified base.
  source 1..13: mol_type = other RNA
acccaccaactca

SEQ ID NO: 341 - RNA, 13 nt, synthetic construct
  misc_feature 1..13: note = Synthetic sequence
  misc_feature 1..13: note = U can be replaced by T. Any base can be replaced with a modified base.
  source 1..13: mol_type = other RNA
tacccaccaactc

SEQ ID NO: 342 - RNA, 13 nt, synthetic construct
  misc_feature 1..13: note = Synthetic sequence
  misc_feature 1..13: note = U can be replaced by T. Any base can be replaced with a modified base.
  source 1..13: mol_type = other RNA
ctacccaccaact

SEQ ID NO: 343 - RNA, 13 nt, synthetic construct
  misc_feature 1..13: note = Synthetic sequence
  misc_feature 1..13: note = U can be replaced by T. Any base can be replaced with a modified base.
  source 1..13: mol_type = other RNA
tctacccaccaac

SEQ ID NO: 344 - RNA, 13 nt, synthetic construct
  misc_feature 1..13: note = Synthetic sequence
  misc_feature 1..13: note = U can be replaced by T. Any base can be replaced with a modified base.
  source 1..13: mol_type = other RNA
atctacccaccaa

SEQ ID NO: 345 - RNA, 13 nt, synthetic construct
  misc_feature 1..13: note = Synthetic sequence
  misc_feature 1..13: note = U can be replaced by T. Any base can be replaced with a modified base.
  source 1..13: mol_type = other RNA
aatctacccacca

SEQ ID NO: 346 - RNA, 13 nt, synthetic construct
  misc_feature 1..13: note = Synthetic sequence
  misc_feature 1..13: note = U can be replaced by T. Any base can be replaced with a modified base.
  source 1..13: mol_type = other RNA
gaatctacccacc

SEQ ID NO: 347 - RNA, 13 nt, synthetic construct
  misc_feature 1..13: note = Synthetic sequence
  source 1..13: mol_type = other RNA
cgaatctacccac

SEQ ID NO: 348 - RNA, 13 nt, synthetic construct
  misc_feature 1..13: note = Synthetic sequence
  source 1..13: mol_type = other RNA
acgaatctaccca

SEQ ID NO: 349 - RNA, 13 nt, synthetic construct
  misc_feature 1..13: note = Synthetic sequence
  misc_feature 1..13: note = U can be replaced by T. Any base can be replaced with a modified base.
  source 1..13: mol_type = other RNA
cacgaatctaccc

SEQ ID NO: 350 - RNA, 13 nt, synthetic construct
  misc_feature 1..13: note = Synthetic sequence
  misc_feature 1..13: note = U can be replaced by T. Any base can be replaced with a modified base.
  source 1..13: mol_type = other RNA
ccacgaatctacc

SEQ ID NO: 351 - RNA, 13 nt, synthetic construct
  misc_feature 1..13: note = Synthetic sequence
  misc_feature 1..13: note = U can be replaced by T. Any base can be replaced with a modified base.
  source 1..13: mol_type = other RNA
gccacgaatctac

SEQ ID NO: 352 - RNA, 13 nt, synthetic construct
  misc_feature 1..13: note = Synthetic sequence
  misc_feature 1..13: note = U can be replaced by T. Any base can be replaced with a modified base.
  source 1..13: mol_type = other RNA
agccacgaatcta

SEQ ID NO: 353 - RNA, 13 nt, synthetic construct
  misc_feature 1..13: note = Synthetic sequence
  misc_feature 1..13: note = U can be replaced by T. Any base can be replaced with a modified base.
  source 1..13: mol_type = other RNA
cagccactcacaa

SEQ ID NO: 354 - RNA, 13 nt, synthetic construct
  misc_feature 1..13: note = Synthetic sequence
  misc_feature 1..13: note = U can be replaced by T. Any base can be replaced with a modified base.
  source 1..13: mol_type = other RNA
ccagccactcaca

SEQ ID NO: 355 - RNA, 13 nt, synthetic construct
  misc_feature 1..13: note = SEQ ID NO 355
  misc_feature 1..13: note = U can be replaced by T. Any base can be replaced with a modified base.
  source 1..13: mol_type = other RNA
accagccactcac

SEQ ID NO: 356 - RNA, 13 nt, synthetic construct
  misc_feature 1..13: note = Synthetic sequence
  misc_feature 1..13: note = U can be replaced by T. Any base can be replaced with a modified base.
  source 1..13: mol_type = other RNA
caccagccactca

SEQ ID NO: 357 - RNA, 13 nt, synthetic construct
  misc_feature 1..13: note = Synthetic sequence
  misc_feature 1..13: note = U can be replaced by T. Any base can be replaced with a modified base.
  source 1..13: mol_type = other RNA
ccaccagccactc

SEQ ID NO: 358 - RNA, 13 nt, synthetic construct
  misc_feature 1..13: note = Synthetic sequence
  misc_feature 1..13: note = U can be replaced by T. Any base can be replaced with a modified base.
  source 1..13: mol_type = other RNA
tccaccagccact

SEQ ID NO: 359 - RNA, 13 nt, synthetic construct
  misc_feature 1..13: note = Synthetic sequence
  misc_feature 1..13: note = U can be replaced by T. Any base can be replaced with a modified base.
  source 1..13: mol_type = other RNA
gtccaccagccac

SEQ ID NO: 360 - RNA, 13 nt, synthetic construct
  misc_feature 1..13: note = Synthetic sequence
  misc_feature 1..13: note = U can be replaced by T. Any base can be replaced with a modified base.
  source 1..13: mol_type = other RNA
tgtccaccagcca

SEQ ID NO: 361 - RNA, 13 nt, synthetic construct
  misc_feature 1..13: note = Synthetic sequence
  misc_feature 1..13: note = U can be replaced by T. Any base can be replaced with a modified base.
  source 1..13: mol_type = other RNA
ctgtccaccagcc

SEQ ID NO: 362 - RNA, 13 nt, synthetic construct
  misc_feature 1..13: note = Synthetic sequence
  misc_feature 1..13: note = U can be replaced by T. Any base can be replaced with a modified base.
  source 1..13: mol_type = other RNA
tctgtccaccagc

SEQ ID NO: 363 - RNA, 13 nt, synthetic construct
  misc_feature 1..13: note = Synthetic sequence
  misc_feature 1..13: note = U can be replaced by T. Any base can be replaced with a modified base.
  source 1..13: mol_type = other RNA
gtctgtccaccag

SEQ ID NO: 364 - RNA, 13 nt, synthetic construct
  misc_feature 1..13: note = Synthetic sequence
  misc_feature 1..13: note = U can be replaced by T. Any base can be replaced with a modified base.
  source 1..13: mol_type = other RNA
cgtctgtccacca

SEQ ID NO: 365 - RNA, 13 nt, synthetic construct
  misc_feature 1..13: note = Synthetic sequence
  misc_feature 1..13: note = U can be replaced by T. Any base can be replaced with a modified base.
  source 1..13: mol_type = other RNA
tcgtctgtccacc

SEQ ID NO: 366 - RNA, 13 nt, synthetic construct
  misc_feature 1..13: note = Synthetic sequence
  misc_feature 1..13: note = U can be replaced by T. Any base can be replaced with a modified base.
  source 1..13: mol_type = other RNA
ttcgtctgtccac

SEQ ID NO: 367 - RNA, 13 nt, synthetic construct
  misc_feature 1..13: note = Synthetic sequence
  misc_feature 1..13: note = U can be replaced by T. Any base can be replaced with a modified base.
  source 1..13: mol_type = other RNA
tttcgtctgtcca

SEQ ID NO: 368 - RNA, 13 nt, synthetic construct
  misc_feature 1..13: note = Synthetic sequence
  misc_feature 1..13: note = U can be replaced by T. Any base can be replaced with a modified base.
  source 1..13: mol_type = other RNA
ttttcgtctgtcc

SEQ ID NO: 369 - RNA, 13 nt, synthetic construct
  misc_feature 1..13: note = Synthetic sequence
  misc_feature 1..13: note = U can be replaced by T. Any base can be replaced with a modified base.
  source 1..13: mol_type = other RNA
tttttcgtctgtc

SEQ ID NO: 370 - RNA, 13 nt, synthetic construct
  misc_feature 1..13: note = Synthetic sequence
  misc_feature 1..13: note = U can be replaced by T. Any base can be replaced with a modified base.
  source 1..13: mol_type = other RNA
atttttcgtctgt

SEQ ID NO: 371 - RNA, 13 nt, synthetic construct
  misc_feature 1..13: note = Synthetic sequence
  misc_feature 1..13: note = U can be replaced by T. Any base can be replaced with a modified base.
  source 1..13: mol_type = other RNA
catttttcgtctg

SEQ ID NO: 372 - RNA, 13 nt, synthetic construct
  misc_feature 1..13: note = Synthetic sequence
  misc_feature 1..13: note = U can be replaced by T. Any base can be replaced with a modified base.
  source 1..13: mol_type = other RNA
ccatttttcgtct

SEQ ID NO: 373 - RNA, 13 nt, synthetic construct
  misc_feature 1..13: note = Synthetic sequence
  misc_feature 1..13: note = U can be replaced by T. Any base can be replaced with a modified base.
  source 1..13: mol_type = other RNA
tccatttttcgtc

SEQ ID NO: 374 - RNA, 13 nt, synthetic construct
  misc_feature 1..13: note = Synthetic sequence
  misc_feature 1..13: note = U can be replaced by T. Any base can be replaced with a modified base.
  source 1..13: mol_type = other RNA
atccatttttcgt

SEQ ID NO: 375 - RNA, 13 nt, synthetic construct
  misc_feature 1..13: note = Synthetic sequence
  misc_feature 1..13: note = U can be replaced by T. Any base can be replaced with a modified base.
  source 1..13: mol_type = other RNA
catccatttttcg

SEQ ID NO: 376 - RNA, 13 nt, synthetic construct
  misc_feature 1..13: note = Synthetic sequence
  misc_feature 1..13: note = U can be replaced by T. Any base can be replaced with a modified base.
  source 1..13: mol_type = other RNA
ccatccatttttc

SEQ ID NO: 377 - RNA, 13 nt, synthetic construct
  misc_feature 1..13: note = Synthetic sequence
  misc_feature 1..13: note = U can be replaced by T. Any base can be replaced with a modified base.
  source 1..13: mol_type = other RNA
accatccattttt

SEQ ID NO: 378 - RNA, 13 nt, synthetic construct
  misc_feature 1..13: note = Synthetic sequence
  misc_feature 1..13: note = U can be replaced by T. Any base can be replaced with a modified base.
  source 1..13: mol_type = other RNA
cccatccattttt

SEQ ID NO: 379 - RNA, 13 nt, synthetic construct
  misc_feature 1..13: note = Synthetic sequence
  misc_feature 1..13: note = U can be replaced by T. Any base can be replaced with a modified base.
  source 1..13: mol_type = other RNA
aaccatccatttt

SEQ ID NO: 380 - RNA, 13 nt, synthetic construct
  misc_feature 1..13: note = Synthetic sequence
  misc_feature 1..13: note = U can be replaced by T. Any base can be replaced with a modified base.
  source 1..13: mol_type = other RNA
acccatccatttt

SEQ ID NO: 381 - RNA, 13 nt, synthetic construct
  misc_feature 1..13: note = Synthetic sequence
  misc_feature 1..13: note = U can be replaced by T. Any base can be replaced with a modified base.
  source 1..13: mol_type = other RNA
caaccatccattt

SEQ ID NO: 382 - RNA, 13 nt, synthetic construct
  misc_feature 1..13: note = Synthetic sequence
  misc_feature 1..13: note = U can be replaced by T. Any base can be replaced with a modified base.
  source 1..13: mol_type = other RNA
cacccatccattt

SEQ ID NO: 383 - RNA, 13 nt, synthetic construct
  misc_feature 1..13: note = Synthetic sequence
  misc_feature 1..13: note = U can be replaced by T. Any base can be replaced with a modified base.
  source 1..13: mol_type = other RNA
ccaaccatccatt

SEQ ID NO: 384 - RNA, 13 nt, synthetic construct
  misc_feature 1..13: note = Synthetic sequence
  misc_feature 1..13: note = U can be replaced by T. Any base can be replaced with a modified base.
  source 1..13: mol_type = other RNA
ccacccatccatt

SEQ ID NO: 385 - RNA, 13 nt, synthetic construct
  misc_feature 1..13: note = Synthetic sequence
  misc_feature 1..13: note = U can be replaced by T. Any base can be replaced with a modified base.
  source 1..13: mol_type = other RNA
tccaaccatccat

SEQ ID NO: 386 - RNA, 13 nt, synthetic construct
  misc_feature 1..13: note = Synthetic sequence
  misc_feature 1..13: note = U can be replaced by T. Any base can be replaced with a modified base.
  source 1..13: mol_type = other RNA
tccacccatccat

SEQ ID NO: 387 - RNA, 13 nt, synthetic construct
  misc_feature 1..13: note = Synthetic sequence
  misc_feature 1..13: note = U can be replaced by T. Any base can be replaced with a modified base.
  source 1..13: mol_type = other RNA
atccaaccatcca

SEQ ID NO: 388 - RNA, 13 nt, synthetic construct
  misc_feature 1..13: note = Synthetic sequence
  misc_feature 1..13: note = U can be replaced by T. Any base can be replaced with a modified base.
  source 1..13: mol_type = other RNA
atccacccatcca

SEQ ID NO: 389 - RNA, 13 nt, synthetic construct
  misc_feature 1..13: note = Synthetic sequence
  misc_feature 1..13: note = U can be replaced by T. Any base can be replaced with a modified base.
  source 1..13: mol_type = other RNA
tatccaaccatcc

SEQ ID NO: 390 - RNA, 13 nt, synthetic construct
  misc_feature 1..13: note = Synthetic sequence
  misc_feature 1..13: note = U can be replaced by T. Any base can be replaced with a modified base.
  source 1..13: mol_type = other RNA
tatccacccatcc

SEQ ID NO: 391 - RNA, 13 nt, synthetic construct
  misc_feature 1..13: note = Synthetic sequence
  misc_feature 1..13: note = U can be replaced by T. Any base can be replaced with a modified base.
  source 1..13: mol_type = other RNA
ttatccaaccatc

SEQ ID NO: 392 - RNA, 13 nt, synthetic construct
  misc_feature 1..13: note = Synthetic sequence
  misc_feature 1..13: note = U can be replaced by T. Any base can be replaced with a modified base.
  source 1..13: mol_type = other RNA
ttatccacccatc

SEQ ID NO: 393 - RNA, 13 nt, synthetic construct
  misc_feature 1..13: note = Synthetic sequence
  misc_feature 1..13: note = U can be replaced by T. Any base can be replaced with a modified base.
  source 1..13: mol_type = other RNA
tttatccaaccat

SEQ ID NO: 394 - RNA, 13 nt, synthetic construct
  misc_feature 1..13: note = Synthetic sequence
  misc_feature 1..13: note = U can be replaced by T. Any base can be replaced with a modified base.
  source 1..13: mol_type = other RNA
tttatccacccat

SEQ ID NO: 395 - RNA, 13 nt, synthetic construct
  misc_feature 1..13: note = Synthetic sequence
  misc_feature 1..13: note = U can be replaced by T. Any base can be replaced with a modified base.
  source 1..13: mol_type = other RNA
atttatccaacca

SEQ ID NO: 396 - RNA, 13 nt, synthetic construct
  misc_feature 1..13: note = Synthetic sequence
  misc_feature 1..13: note = U can be replaced by T. Any base can be replaced with a modified base.
  source 1..13: mol_type = other RNA
atttatccaccca

SEQ ID NO: 397 - RNA, 13 nt, synthetic construct
  misc_feature 1..13: note = Synthetic sequence
  misc_feature 1..13: note = U can be replaced by T. Any base can be replaced with a modified base.
  source 1..13: mol_type = other RNA
aatttatccaacc

SEQ ID NO: 398 - RNA, 13 nt, synthetic construct
  misc_feature 1..13: note = Synthetic sequence
  misc_feature 1..13: note = U can be replaced by T. Any base can be replaced with a modified base.
  source 1..13: mol_type = other RNA
aatttatccaccc

SEQ ID NO: 399 - RNA, 13 nt, synthetic construct
  misc_feature 1..13: note = Synthetic sequence
  misc_feature 1..13: note = U can be replaced by T. Any base can be replaced with a modified base.
  source 1..13: mol_type = other RNA
caatttatccaac

SEQ ID NO: 400 - RNA, 13 nt, synthetic construct
  misc_feature 1..13: note = Synthetic sequence
  misc_feature 1..13: note = U can be replaced by T. Any base can be replaced with a modified base.
  source 1..13: mol_type = other RNA
caatttatccacc

SEQ ID NO: 401 - RNA, 13 nt, synthetic construct
  misc_feature 1..13: note = Synthetic sequence
  misc_feature 1..13: note = U can be replaced by T. Any base can be replaced with a modified base.
  source 1..13: mol_type = other RNA
tcaatttatccaa

SEQ ID NO: 402 - RNA, 13 nt, synthetic construct
  misc_feature 1..13: note = Synthetic sequence
  misc_feature 1..13: note = U can be replaced by T. Any base can be replaced with a modified base.
  source 1..13: mol_type = other RNA
tcaatttatccac

SEQ ID NO: 403 - RNA, 13 nt, synthetic construct
  misc_feature 1..13: note = Synthetic sequence
  misc_feature 1..13: note = U can be replaced by T. Any base can be replaced with a modified base.
  source 1..13: mol_type = other RNA
atcaatttatcca

SEQ ID NO: 404 - RNA, 13 nt, synthetic construct
  misc_feature 1..13: note = Synthetic sequence
  misc_feature 1..13: note = U can be replaced by T. Any base can be replaced with a modified base.
  source 1..13: mol_type = other RNA
catcaatttatcc

SEQ ID NO: 405 - RNA, 13 nt, synthetic construct
  misc_feature 1..13: note = Synthetic sequence
  misc_feature 1..13: note = U can be replaced by T. Any base can be replaced with a modified base.
  source 1..13: mol_type = other RNA
ccatcaatttatc

SEQ ID NO: 406 - RNA, 13 nt, synthetic construct
  misc_feature 1..13: note = Synthetic sequence
  misc_feature 1..13: note = U can be replaced by T. Any base can be replaced with a modified base.
  source 1..13: mol_type = other RNA
cccatcaatttat

SEQ ID NO: 407 - RNA, 13 nt, synthetic construct
  misc_feature 1..13: note = Synthetic sequence
  misc_feature 1..13: note = U can be replaced by T. Any base can be replaced with a modified base.
  source 1..13: mol_type = other RNA
acccatcaattta

SEQ ID NO: 408 - RNA, 13 nt, synthetic construct
  misc_feature 1..13: note = Synthetic sequence
  misc_feature 1..13: note = U can be replaced by T. Any base can be replaced with a modified base.
  source 1..13: mol_type = other RNA
cacccatcaattt

SEQ ID NO: 409 - RNA, 13 nt, synthetic construct
  misc_feature 1..13: note = Synthetic sequence
  misc_feature 1..13: note = U can be replaced by T. Any base can be replaced with a modified base.
  source 1..13: mol_type = other RNA
ccacccatcaatt

SEQ ID NO: 410 - RNA, 13 nt, synthetic construct
  misc_feature 1..13: note = Synthetic sequence
  misc_feature 1..13: note = U can be replaced by T. Any base can be replaced with a modified base.
  source 1..13: mol_type = other RNA
tccacccatcaat

SEQ ID NO: 411 - RNA, 13 nt, synthetic construct
  misc_feature 1..13: note = Synthetic sequence
  misc_feature 1..13: note = U can be replaced by T. Any base can be replaced with a modified base.
  source 1..13: mol_type = other RNA
atccacccatcaa

SEQ ID NO: 412 - RNA, 13 nt, synthetic construct
  misc_feature 1..13: note = Synthetic sequence
  misc_feature 1..13: note = U can be replaced by T. Any base can be replaced with a modified base.
  source 1..13: mol_type = other RNA
catccacccatca

SEQ ID NO: 413 - RNA, 13 nt, synthetic construct
  misc_feature 1..13: note = Synthetic sequence
  misc_feature 1..13: note = U can be replaced by T. Any base can be replaced with a modified base.
  source 1..13: mol_type = other RNA
ccatccacccatc

SEQ ID NO: 414 - RNA, 13 nt, synthetic construct
  misc_feature 1..13: note = Synthetic sequence
  misc_feature 1..13: note = U can be replaced by T. Any base can be replaced with a modified base.
  source 1..13: mol_type = other RNA
tccatccacccat

SEQ ID NO: 415 - RNA, 13 nt, synthetic construct
  misc_feature 1..13: note = Synthetic sequence
  misc_feature 1..13: note = U can be replaced by T. Any base can be replaced with a modified base.
  source 1..13: mol_type = other RNA
atccatccaccca

SEQ ID NO: 416 - RNA, 13 nt, synthetic construct
  misc_feature 1..13: note = Synthetic sequence
  misc_feature 1..13: note = U can be replaced by T. Any base can be replaced with a modified base.
  source 1..13: mol_type = other RNA
catccatccaccc

SEQ ID NO: 417 - RNA, 13 nt, synthetic construct
  misc_feature 1..13: note = Synthetic sequence
  misc_feature 1..13: note = U can be replaced by T. Any base can be replaced with a modified base.
  source 1..13: mol_type = other RNA
ccatccatccacc

SEQ ID NO: 418 - RNA, 13 nt, synthetic construct
  misc_feature 1..13: note = Synthetic sequence
  misc_feature 1..13: note = U can be replaced by T. Any base can be replaced with a modified base.
  source 1..13: mol_type = other RNA
accatccatccac

SEQ ID NO: 419 - RNA, 13 nt, synthetic construct
  misc_feature 1..13: note = Synthetic sequence
  misc_feature 1..13: note = U can be replaced by T. Any base can be replaced with a modified base.
  source 1..13: mol_type = other RNA
aaccatccatcca

SEQ ID NO: 420 - RNA, 13 nt, synthetic construct
  misc_feature 1..13: note = Synthetic sequence
  misc_feature 1..13: note = U can be replaced by T. Any base can be replaced with a modified base.
  source 1..13: mol_type = other RNA
caaccatccatcc

SEQ ID NO: 421 - RNA, 13 nt, synthetic construct
  misc_feature 1..13: note = Synthetic sequence
  misc_feature 1..13: note = U can be replaced by T. Any base can be replaced with a modified base.
  source 1..13: mol_type = other RNA
ccaaccatccatc

SEQ ID NO: 422 - RNA, 13 nt, synthetic construct
  misc_feature 1..13: note = Synthetic sequence
  misc_feature 1..13: note = U can be replaced by T. Any base can be replaced with a modified base.
  source 1..13: mol_type = other RNA
accaaccatccat

SEQ ID NO: 423 - RNA, 13 nt, synthetic construct
  misc_feature 1..13: note = Synthetic sequence
  misc_feature 1..13: note = U can be replaced by T. Any base can be replaced with a modified base.
  source 1..13: mol_type = other RNA
aaccaaccatcca

SEQ ID NO: 424 - RNA, 13 nt, synthetic construct
  misc_feature 1..13: note = Synthetic sequence
  misc_feature 1..13: note = U can be replaced by T. Any base can be replaced with a modified base.
  source 1..13: mol_type = other RNA
caaccaaccatcc

SEQ ID NO: 425 - RNA, 13 nt, synthetic construct
  misc_feature 1..13: note = Synthetic sequence
  misc_feature 1..13: note = U can be replaced by T. Any base can be replaced with a modified base.
  source 1..13: mol_type = other RNA
acaaccaaccatc

SEQ ID NO: 426 - RNA, 13 nt, synthetic construct
  misc_feature 1..13: note = Synthetic sequence
  misc_feature 1..13: note = U can be replaced by T. Any base can be replaced with a modified base.
  source 1..13: mol_type = other RNA
tacaaccaaccat

SEQ ID NO: 427 - RNA, 13 nt, synthetic construct
  misc_feature 1..13: note = Synthetic sequence
  misc_feature 1..13: note = U can be replaced by T. Any base can be replaced with a modified base.
  source 1..13: mol_type = other RNA
tccgcaacttaat

SEQ ID NO: 428 - RNA, 13 nt, synthetic construct
  misc_feature 1..13: note = Synthetic sequence
  misc_feature 1..13: note = U can be replaced by T. Any base can be replaced with a modified base.
  source 1..13: mol_type = other RNA
atccgcaacttaa

SEQ ID NO: 429 - RNA, 13 nt, synthetic construct
  misc_feature 1..13: note = Synthetic sequence
  misc_feature 1..13: note = U can be replaced by T. Any base can be replaced with a modified base.
  source 1..13: mol_type = other RNA
gatccgcaactta

SEQ ID NO: 430 - RNA, 13 nt, synthetic construct
  misc_feature 1..13: note = Synthetic sequence
  misc_feature 1..13: note = U can be replaced by T. Any base can be replaced with a modified base.
  source 1..13: mol_type = other RNA
tgatccgcaactt

SEQ ID NO: 431 - RNA, 13 nt, synthetic construct
  misc_feature 1..13: note = Synthetic sequence
  misc_feature 1..13: note = U can be replaced by T. Any base can be replaced with a modified base.
  source 1..13: mol_type = other RNA
ttgatccgcaact

SEQ ID NO: 432 - RNA, 13 nt, synthetic construct
  misc_feature 1..13: note = Synthetic sequence
  misc_feature 1..13: note = U can be replaced by T. Any base can be replaced with a modified base.
  source 1..13: mol_type = other RNA
attgatccgcaac

SEQ ID NO: 433 - RNA, 13 nt, synthetic construct
  misc_feature 1..13: note = Synthetic sequence
  misc_feature 1..13: note = U can be replaced by T. Any base can be replaced with a modified base.
  source 1..13: mol_type = other RNA
cattgatccgcaa

SEQ ID NO: 434 - RNA, 13 nt, synthetic construct
  misc_feature 1..13: note = Synthetic sequence
  misc_feature 1..13
  source 1..13: mol_type = other RNA
acattgatccgca

SEQ ID NO: 435 - RNA, 13 nt, synthetic construct
  misc_feature 1..13: note = Synthetic sequence
  misc_feature 1..13: note = U can be replaced by T. Any base can be replaced with a modified base.
  source 1..13: mol_type = other RNA
tacattgatccgc

SEQ ID NO: 436 - RNA, 13 nt, synthetic construct
  misc_feature 1..13: note = Synthetic sequence
  misc_feature 1..13: note = U can be replaced by T. Any base can be replaced with a modified base.
  source 1..13: mol_type = other RNA
atacattgatccg

SEQ ID NO: 437 - RNA, 13 nt, synthetic construct
  misc_feature 1..13: note = Synthetic sequence
  misc_feature 1..13: note = U can be replaced by T. Any base can be replaced with a modified base.
  source 1..13: mol_type = other RNA
catacattgatcc

SEQ ID NO: 438 - RNA, 13 nt, synthetic construct
  misc_feature 1..13: note = Synthetic sequence
  misc_feature 1..13: note = U can be replaced by T. Any base can be replaced with a modified base.
  source 1..13: mol_type = other RNA
ccatacattgatc

SEQ ID NO: 439 - RNA, 13 nt, synthetic construct
  misc_feature 1..13: note = Synthetic sequence
  misc_feature 1..13: note = U can be replaced by T. Any base can be replaced with a modified base.
  source 1..13: mol_type = other RNA
cccatacattgat

SEQ ID NO: 440 - RNA, 13 nt, synthetic construct
  misc_feature 1..13: note = Synthetic sequence
  misc_feature 1..13: note = U can be replaced by T. Any base can be replaced with a modified base.
  source 1..13: mol_type = other RNA
tcccatacattga

SEQ ID NO: 441 - RNA, 13 nt, synthetic construct
  misc_feature 1..13: note = Synthetic sequence
  misc_feature 1..13: note = U can be replaced by T. Any base can be replaced with a modified base.
  source 1..13: mol_type = other RNA
atcccatacattg

SEQ ID NO: 442 - RNA, 13 nt, synthetic construct
  misc_feature 1..13: note = Synthetic sequence
  misc_feature 1..13: note = U can be replaced by T. Any base can be replaced with a modified base.
  source 1..13: mol_type = other RNA
catcccatacatt

SEQ ID NO: 443 - RNA, 13 nt, synthetic construct
  misc_feature 1..13: note = Synthetic sequence
  misc_feature 1..13: note = U can be replaced by T. Any base can be replaced with a modified base.
  source 1..13: mol_type = other RNA
ccatcccatacat

SEQ ID NO: 444 - RNA, 13 nt, synthetic construct
  misc_feature 1..13: note = Synthetic sequence
  misc_feature 1..13: note = U can be replaced by T. Any base can be replaced with a modified base.
  source 1..13: mol_type = other RNA
tccatcccataca

SEQ ID NO: 445 - RNA, 13 nt, synthetic construct
  misc_feature 1..13: note = Synthetic sequence
  misc_feature 1..13: note = U can be replaced by T. Any base can be replaced with a modified base.
  source 1..13: mol_type = other RNA
atccatcccatac

SEQ ID NO: 446 - RNA, 13 nt, synthetic construct
  misc_feature 1..13: note = Synthetic sequence
  misc_feature 1..13: note = U can be replaced by T. Any base can be replaced with a modified base.
  source 1..13: mol_type = other RNA
catccatcccata

SEQ ID NO: 447 - RNA, 13 nt, synthetic construct
  misc_feature 1..13: note = Synthetic sequence
  misc_feature 1..13: note = U can be replaced by T. Any base can be replaced with a modified base.
  source 1..13: mol_type = other RNA
tcatccatcccat

SEQ ID NO: 448 - RNA, 13 nt, synthetic construct
  misc_feature 1..13: note = Synthetic sequence
  misc_feature 1..13: note = U can be replaced by T. Any base can be replaced with a modified base.
  source 1..13: mol_type = other RNA
ttcatccatccca

SEQ ID NO: 449 - RNA, 13 nt, synthetic construct
  misc_feature 1..13: note = Synthetic sequence
  misc_feature 1..13: note = U can be replaced by T. Any base can be replaced with a modified base.
  source 1..13: mol_type = other RNA
attcatccatccc

SEQ ID NO: 450 - RNA, 13 nt, synthetic construct
  misc_feature 1..13: note = Synthetic sequence
  misc_feature 1..13: note = U can be replaced by T. Any base can be replaced with a modified base.
  source 1..13: mol_type = other RNA
cattcatccatcc

SEQ ID NO: 451 - RNA, 13 nt, synthetic construct
  misc_feature 1..13: note = Synthetic sequence
  misc_feature 1..13: note = U can be replaced by T. Any base can be replaced with a modified base.
  source 1..13: mol_type = other RNA
ccattcatccatc

SEQ ID NO: 452 - RNA, 13 nt, synthetic construct
  misc_feature 1..13: note = Synthetic sequence
  misc_feature 1..13: note = U can be replaced by T. Any base can be replaced with a modified base.
  source 1..13: mol_type = other RNA
tccattcatccat

SEQ ID NO: 453 - RNA, 13 nt, synthetic construct
  misc_feature 1..13: note = Synthetic sequence
  misc_feature 1..13: note = U can be replaced by T. Any base can be replaced with a modified base.
  source 1..13: mol_type = other RNA
atccattcatcca

SEQ ID NO: 454 - RNA, 12 nt, synthetic construct
  misc_feature 1..12: note = Synthetic sequence
  misc_feature 1..12: note = U can be replaced by T. Any base can be replaced with a modified base.
  source 1..12: mol_type = other RNA
catccattcatc

SEQ ID NO: 455 - RNA, 13 nt, synthetic construct
  misc_feature 1..13: note = Synthetic sequence
  misc_feature 1..13: note = U can be replaced by T. Any base can be replaced with a modified base.
  source 1..13: mol_type = other RNA
ccatccattcatc

SEQ ID NO: 456 - RNA, 13 nt, synthetic construct
  misc_feature 1..13: note = Synthetic sequence
  misc_feature 1..13: note = U can be replaced by T. Any base can be replaced with a modified base.
  source 1..13: mol_type = other RNA
tccatccattcat

SEQ ID NO: 457 - RNA, 13 nt, synthetic construct
  misc_feature 1..13: note = Synthetic sequence
  misc_feature 1..13: note = U can be replaced by T. Any base can be replaced with a modified base.
  source 1..13: mol_type = other RNA
atccatccattca

SEQ ID NO: 458 - RNA, 13 nt, synthetic construct
  misc_feature 1..13: note = Synthetic sequence
  misc_feature 1..13: note = U can be replaced by T. Any base can be replaced with a modified base.
  source 1..13: mol_type = other RNA
catccatccattc

SEQ ID NO: 459 - RNA, 13 nt, synthetic construct
  misc_feature 1..13: note = Synthetic sequence
  misc_feature 1..13: note = U can be replaced by T. Any base can be replaced with a modified base.
  source 1..13: mol_type = other RNA
ccatccatccatt

SEQ ID NO: 460 - RNA, 13 nt, synthetic construct
  misc_feature 1..13: note = Synthetic sequence
  misc_feature 1..13: note = U can be replaced by T. Any base can be replaced with a modified base.
  source 1..13: mol_type = other RNA
tccatccatccat

SEQ ID NO: 461 - RNA, 13 nt, synthetic construct
  misc_feature 1..13: note = Synthetic sequence
  misc_feature 1..13: note = U can be replaced by T. Any base can be replaced with a modified base.
  source 1..13: mol_type = other RNA
atccatccatcca

SEQ ID NO: 462 - RNA, 13 nt, synthetic construct
  misc_feature 1..13: note = Synthetic sequence
  misc_feature 1..13: note = U can be replaced by T. Any base can be replaced with a modified base.
  source 1..13: mol_type = other RNA
catccatccatcc

SEQ ID NO: 463 - RNA, 13 nt, synthetic construct
  misc_feature 1..13: note = Synthetic sequence
  misc_feature 1..13: note = U can be replaced by T. Any base can be replaced with a modified base.
  source 1..13: mol_type = other RNA
ccatccatccatc

SEQ ID NO: 464 - RNA, 13 nt, synthetic construct
  misc_feature 1..13: note = Synthetic sequence
  misc_feature 1..13: note = U can be replaced by T. Any base can be replaced with a modified base.
  source 1..13: mol_type = other RNA
acatccatccatc

SEQ ID NO: 465 - RNA, 13 nt, synthetic construct
  misc_feature 1..13: note = Synthetic sequence
  misc_feature 1..13: note = U can be replaced by T. Any base can be replaced with a modified base.
  source 1..13: mol_type = other RNA
cacatccatccat

SEQ ID NO: 466 - RNA, 13 nt, synthetic construct
  misc_feature 1..13: note = Synthetic sequence
  misc_feature 1..13: note = U can be replaced by T. Any base can be replaced with a modified base.
  source 1..13: mol_type = other RNA
acacatccatcca

SEQ ID NO: 467 - RNA, 13 nt, synthetic construct
  misc_feature 1..13: note = Synthetic sequence
  misc_feature 1..13: note = U can be replaced by T. Any base can be replaced with a modified base.
  source 1..13: mol_type = other RNA
cacacatccatcc

SEQ ID NO: 468 - RNA, 13 nt, synthetic construct
  misc_feature 1..13: note = Synthetic sequence
  misc_feature 1..13: note = U can be replaced by T. Any base can be replaced with a modified base.
  source 1..13: mol_type = other RNA
ccacacatccatc

SEQ ID NO: 469 - RNA, 13 nt, synthetic construct
  misc_feature 1..13: note = Synthetic sequence
  misc_feature 1..13: note = U can be replaced by T. Any base can be replaced with a modified base.
  source 1..13: mol_type = other RNA
accacacatccat

SEQ ID NO: 470 - RNA, 13 nt, synthetic construct
  misc_feature 1..13: note = Synthetic sequence
  misc_feature 1..13: note = U can be replaced by T. Any base can be replaced with a modified base.
  source 1..13: mol_type = other RNA
aaccacacatcca

SEQ ID NO: 471 - RNA, 13 nt, synthetic construct
  misc_feature 1..13: note = Synthetic sequence
  misc_feature 1..13: note = U can be replaced by T. Any base can be replaced with a modified base.
  source 1..13: mol_type = other RNA
caaccacacatcc

SEQ ID NO: 472 - RNA, 13 nt, synthetic construct
  misc_feature 1..13: note = Synthetic sequence
  misc_feature 1..13: note = U can be replaced by T. Any base can be replaced with a modified base.
  source 1..13: mol_type = other RNA
tcaaccacacatc

SEQ ID NO: 473 - RNA, 13 nt, synthetic construct
  misc_feature 1..13: note = Synthetic sequence
  misc_feature 1..13: note = U can be replaced by T. Any base can be replaced with a modified base.
  source 1..13: mol_type = other RNA
ttcaaccacacat

SEQ ID NO: 474 - RNA, 13 nt, synthetic construct
  misc_feature 1..13: note = Synthetic sequence
  misc_feature 1..13: note = U can be replaced by T. Any base can be replaced with a modified base.
  source 1..13: mol_type = other RNA
attcaaccacaca

SEQ ID NO: 475 - RNA, 13 nt, synthetic construct
  misc_feature 1..13: note = Synthetic sequence
  misc_feature 1..13: note = U can be replaced by T. Any base can be replaced with a modified base.
  source 1..13: mol_type = other RNA
tctatccagcaat

SEQ ID NO: 476 - RNA, 13 nt, synthetic construct
  misc_feature 1..13: note = Synthetic sequence
  misc_feature 1..13: note = U can be replaced by T. Any base can be replaced with a modified base.
  source 1..13: mol_type = other RNA
atctatccagcaa

SEQ ID NO: 477 - RNA, 13 nt, synthetic construct
  misc_feature 1..13: note = Synthetic sequence
  misc_feature 1..13: note = U can be replaced by T. Any base can be replaced with a modified base.
  source 1..13: mol_type = other RNA
catctatccagca

SEQ ID NO: 478 - RNA, 13 nt, synthetic construct
  misc_feature 1..13: note = Synthetic sequence
  misc_feature 1..13: note = U can be replaced by T. Any base can be replaced with a modified base.
  source 1..13: mol_type = other RNA
tcatctatccagc

SEQ ID NO: 479 - RNA, 13 nt, synthetic construct
  misc_feature 1..13: note = Synthetic sequence
  misc_feature 1..13: note = U can be replaced by T. Any base can be replaced with a modified base.
  source 1..13: mol_type = other RNA
atcatctatccag

SEQ ID NO: 480 - RNA, 13 nt, synthetic construct
  misc_feature 1..13: note = Synthetic sequence
  misc_feature 1..13: note = U can be replaced by T. Any base can be replaced with a modified base.
  source 1..13: mol_type = other RNA
aatcatctatcca

SEQ ID NO: 481 - RNA, 13 nt, synthetic construct
  misc_feature 1..13: note = Synthetic sequence
  misc_feature 1..13: note = U can be replaced by T. Any base can be replaced with a modified base.
  source 1..13: mol_type = other RNA
caatcatctatcc

SEQ ID NO: 482 - RNA, 13 nt, synthetic construct
  misc_feature 1..13: note = Synthetic sequence
  misc_feature 1..13: note = U can be replaced by T. Any base can be replaced with a modified base.
  source 1..13: mol_type = other RNA
tcaatcatctatc

SEQ ID NO: 483 - RNA, 13 nt, synthetic construct
  misc_feature 1..13: note = Synthetic sequence
  misc_feature 1..13: note = U can be replaced by T. Any base can be replaced with a modified base.
  source 1..13: mol_type = other RNA
gtcaatcatctat

SEQ ID NO: 484 - RNA, 13 nt, synthetic construct
  misc_feature 1..13: note = Synthetic sequence
  misc_feature 1..13: note = U can be replaced by T. Any base can be replaced with a modified base.
  source 1..13: mol_type = other RNA
agtcaatcatcta

SEQ ID NO: 485 - RNA, 13 nt, synthetic construct
  misc_feature 1..13: note = Synthetic sequence
  misc_feature 1..13: note = U can be replaced by T. Any base can be replaced with a modified base.
  source 1..13: mol_type = other RNA
cagtcaatcatct

SEQ ID NO: 486 - RNA, 13 nt, synthetic construct
  misc_feature 1..13: note = Synthetic sequence
  misc_feature 1..13: note = U can be replaced by T. Any base can be replaced with a modified base.
  source 1..13: mol_type = other RNA
ccagtcaatcatc

SEQ ID NO: 487 - RNA, 13 nt, synthetic construct
  misc_feature 1..13: note = Synthetic sequence
  misc_feature 1..13: note = U can be replaced by T. Any base can be replaced with a modified base.
  source 1..13: mol_type = other RNA
cccagtcaatcat

SEQ ID NO: 488 - RNA, 13 nt, synthetic construct
  misc_feature 1..13: note = Synthetic sequence
  misc_feature 1..13: note = U can be replaced by T. Any base can be replaced with a modified base.
  source 1..13: mol_type = other RNA
acccagtcaatca

SEQ ID NO: 489 - RNA, 13 nt, synthetic construct
  misc_feature 1..13: note = Synthetic sequence
  misc_feature 1..13: note = U can be replaced by T. Any base can be replaced with a modified base.
  source 1..13: mol_type = other RNA
cacccagtcaatc

SEQ ID NO: 490 - RNA, 13 nt, synthetic construct
  misc_feature 1..13: note = Synthetic sequence
  misc_feature 1..13: note = U can be replaced by T. Any base can be replaced with a modified base.
  source 1..13: mol_type = other RNA
ccacccagtcaat

SEQ ID NO: 491 - RNA, 13 nt, synthetic construct
  misc_feature 1..13: note = Synthetic sequence
  misc_feature 1..13: note = U can be replaced by T. Any base can be replaced with a modified base.
  source 1..13: mol_type = other RNA
tccacccagtcaa

SEQ ID NO: 492 - RNA, 13 nt, synthetic construct
  misc_feature 1..13: note = Synthetic sequence
  misc_feature 1..13: note = U can be replaced by T. Any base can be replaced with a modified base.
  source 1..13: mol_type = other RNA
atccacccagtca

SEQ ID NO: 493 - RNA, 13 nt, synthetic construct
  misc_feature 1..13: note = Synthetic sequence
  misc_feature 1..13: note = U can be replaced by T. Any base can be replaced with a modified base.
  source 1..13: mol_type = other RNA
tatccacccagtc

SEQ ID NO: 494 - RNA, 13 nt, synthetic construct
  misc_feature 1..13: note = Synthetic sequence
  misc_feature 1..13: note = U can be replaced by T. Any base can be replaced with a modified base.
  source 1..13: mol_type = other RNA
ctatccacccagt

SEQ ID NO: 495 - RNA, 13 nt, synthetic construct
  misc_feature 1..13: note = Synthetic sequence
  misc_feature 1..13: note = U can be replaced by T. Any base can be replaced with a modified base.
  source 1..13: mol_type = other RNA
tctatccacccag

SEQ ID NO: 496 - RNA, 13 nt, synthetic construct
  misc_feature 1..13: note = Synthetic sequence
  misc_feature 1..13: note = U can be replaced by T. Any base can be replaced with a modified base.
  source 1..13: mol_type = other RNA
atctatccaccca

SEQ ID NO: 497 - RNA, 13 nt, synthetic construct
  misc_feature 1..13: note = Synthetic sequence
  misc_feature 1..13: note = U can be replaced by T. Any base can be replaced with a modified base.
  source 1..13: mol_type = other RNA
catctatccaccc

SEQ ID NO: 498 - RNA, 13 nt, synthetic construct
  misc_feature 1..13: note = Synthetic sequence
  misc_feature 1..13: note = U can be replaced by T. Any base can be replaced with a modified base.
  source 1..13: mol_type = other RNA
tcatctatccacc

SEQ ID NO: 499 - RNA, 13 nt, synthetic construct
  misc_feature 1..13: note = Synthetic sequence
  misc_feature 1..13: note = U can be replaced by T. Any base can be replaced with a modified base.
  source 1..13: mol_type = other RNA
ttcatctatccac

SEQ ID NO: 500 - RNA, 13 nt, synthetic construct
  misc_feature 1..13: note = Synthetic sequence
  misc_feature 1..13: note = U can be replaced by T. Any base can be replaced with a modified base.
  source 1..13: mol_type = other RNA
tttcatctatcca

SEQ ID NO: 501 - RNA, 13 nt, synthetic construct
  misc_feature 1..13: note = Synthetic sequence
  source 1..13: mol_type = other RNA
atttcatctatcc

SEQ ID NO: 502 - RNA, 13 nt, synthetic construct
  misc_feature 1..13: note = Synthetic sequence
  misc_feature 1..13: note = U can be replaced by T. Any base can be replaced with a modified base.
  source 1..13: mol_type = other RNA
catttcatctatc

SEQ ID NO: 503 - RNA, 13 nt, synthetic construct
  misc_feature 1..13: note = Synthetic sequence
  misc_feature 1..13: note = U can be replaced by T. Any base can be replaced with a modified base.
  source 1..13: mol_type = other RNA
acatttcatctat

SEQ ID NO: 504 - RNA, 13 nt, synthetic construct
  misc_feature 1..13: note = Synthetic sequence
  misc_feature 1..13: note = U can be replaced by T. Any base can be replaced with a modified base.
  source 1..13: mol_type = other RNA
aacatttcatcta

SEQ ID NO: 505 - RNA, 13 nt, synthetic construct
  misc_feature 1..13: note = Synthetic sequence
  misc_feature 1..13: note = U can be replaced by T. Any base can be replaced with a modified base.
  source 1..13: mol_type = other RNA
caacatttcatct

SEQ ID NO: 506 - RNA, 13 nt, synthetic construct
  misc_feature 1..13: note = Synthetic sequence
  misc_feature 1..13: note = U can be replaced by T. Any base can be replaced with a modified base.
  source 1..13: mol_type = other RNA
tctggggcagctt

SEQ ID NO: 507 - RNA, 13 nt, synthetic construct
  misc_feature 1..13: note = Synthetic sequence
  misc_feature 1..13: note = U can be replaced by T. Any base can be replaced with a modified base.
  source 1..13: mol_type = other RNA
gtctggggcagct

SEQ ID NO: 508 - RNA, 13 nt, synthetic construct
  misc_feature 1..13: note = Synthetic sequence
  misc_feature 1..13: note = U can be replaced by T. Any base can be replaced with a modified base.
  source 1..13: mol_type = other RNA
ggtctggggcagc

SEQ ID NO: 509 - RNA, 13 nt, synthetic construct
  misc_feature 1..13: note = Synthetic sequence
  misc_feature 1..13: note = U can be replaced by T. Any base can be replaced with a modified base.
  source 1..13: mol_type = other RNA
gggtctggggcag

SEQ ID NO: 510 - RNA, 13 nt, synthetic construct
  misc_feature 1..13: note = Synthetic sequence
  misc_feature 1..13: note = U can be replaced by T. Any base can be replaced with a modified base.
  source 1..13: mol_type = other RNA
agggtctggggca

SEQ ID NO: 511 - RNA, 13 nt, synthetic construct
  misc_feature 1..13: note = Synthetic sequence
  misc_feature 1..13: note = U can be replaced by T. Any base can be replaced with a modified base.
  source 1..13: mol_type = other RNA
cagggtctggggc

SEQ ID NO: 512 - RNA, 13 nt, synthetic construct
  misc_feature 1..13: note = Synthetic sequence
  misc_feature 1..13: note = U can be replaced by T. Any base can be replaced with a modified base.
  source 1..13: mol_type = other RNA
ccagggtctgggg

SEQ ID NO: 513 - RNA, 13 nt, synthetic construct
  misc_feature 1..13: note = Synthetic sequence
  misc_feature 1..13: note = U can be replaced by T. Any base can be replaced with a modified base.
  source 1..13: mol_type = other RNA
cccagggtctggg

SEQ ID NO: 514 - RNA, 13 nt, synthetic construct
  misc_feature 1..13: note = Synthetic sequence
  misc_feature 1..13: note = U can be replaced by T. Any base can be replaced with a modified base.
  source 1..13: mol_type = other RNA
tcccagggtctgg

SEQ ID NO: 515 - RNA, 13 nt, synthetic construct
  misc_feature 1..13: note = Synthetic sequence
  misc_feature 1..13: note = U can be replaced by T. Any base can be replaced with a modified base.
  source 1..13: mol_type = other RNA
gtcccagggtctg

SEQ ID NO: 516 - RNA, 13 nt, synthetic construct
  misc_feature 1..13: note = Synthetic sequence
  misc_feature 1..13: note = U can be replaced by T. Any base can be replaced with a modified base.
  source 1..13: mol_type = other RNA
ggtcccagggtct

SEQ ID NO: 517 - RNA, 13 nt, synthetic construct
  misc_feature 1..13: note = Synthetic sequence
  misc_feature 1..13: note = U can be replaced by T. Any base can be replaced with a modified base.
  source 1..13: mol_type = other RNA
aggtcccagggtc

SEQ ID NO: 518 - RNA, 13 nt, synthetic construct
  misc_feature 1..13: note = Synthetic sequence
  misc_feature 1..13: note = U can be replaced by T. Any base can be replaced with a modified base.
  source 1..13: mol_type = other RNA
gaggtcccagggt

SEQ ID NO: 519 - RNA, 13 nt, synthetic construct
  misc_feature 1..13: note = Synthetic sequence
  misc_feature 1..13: note = U can be replaced by T. Any base can be replaced with a modified base.
  source 1..13: mol_type = other RNA
agaggtcccaggg

SEQ ID NO: 520 - RNA, 13 nt, synthetic construct
  misc_feature 1..13: note = Synthetic sequence
  misc_feature 1..13: note = U can be replaced by T. Any base can be replaced with a modified base.
  source 1..13: mol_type = other RNA
cagaggtcccagg

SEQ ID NO: 521 - RNA, 13 nt, synthetic construct
  misc_feature 1..13: note = Synthetic sequence
  misc_feature 1..13: note = U can be replaced by T. Any base can be replaced with a modified base.
  source 1..13: mol_type = other RNA
tcagaggtcccag

SEQ ID NO: 522 - RNA, 13 nt, synthetic construct
  misc_feature 1..13: note = Synthetic sequence
  misc_feature 1..13: note = U can be replaced by T. Any base can be replaced with a modified base.
  source 1..13: mol_type = other RNA
gtcagaggtccca

SEQ ID NO: 523 - RNA, 13 nt, synthetic construct
  misc_feature 1..13: note = Synthetic sequence
  misc_feature 1..13: note = U can be replaced by T. Any base can be replaced with a modified base.
  source 1..13: mol_type = other RNA
ggtcagaggtccc

SEQ ID NO: 524 - RNA, 13 nt, synthetic construct
  misc_feature 1..13: note = Synthetic sequence
  misc_feature 1..13: note = U can be replaced by T. Any base can be replaced with a modified base.
  source 1..13: mol_type = other RNA
gggtcagaggtcc

SEQ ID NO: 525 - RNA, 13 nt, synthetic construct
  misc_feature 1..13: note = Synthetic sequence
  misc_feature 1..13: note = U can be replaced by T. Any base can be replaced with a modified base.
  source 1..13: mol_type = other RNA
ggggtcagaggtc

SEQ ID NO: 526 - RNA, 13 nt, synthetic construct
  misc_feature 1..13: note = Synthetic sequence
  misc_feature 1..13: note = U can be replaced by T. Any base can be replaced with a modified base.
  source 1..13: mol_type = other RNA
gggggtcagaggt

SEQ ID NO: 527 - RNA, 13 nt, synthetic construct
  misc_feature 1..13: note = Synthetic sequence
  misc_feature 1..13: note = U can be replaced by T. Any base can be replaced with a modified base.
  source 1..13: mol_type = other RNA
cgggggtcagagg

SEQ ID NO: 528 - RNA, 13 nt, synthetic construct
  misc_feature 1..13: note = Synthetic sequence
  misc_feature 1..13: note = U can be replaced by T. Any base can be replaced with a modified base.
  source 1..13: mol_type = other RNA
ccgggggtcagag

SEQ ID NO: 529 - RNA, 13 nt, synthetic construct
  misc_feature 1..13: note = Synthetic sequence
  misc_feature 1..13: note = U can be replaced by T. Any base can be replaced with a modified base.
  source 1..13: mol_type = other RNA
gccgggggtcaga

SEQ ID NO: 530 - RNA, 13 nt, synthetic construct
  misc_feature 1..13: note = Synthetic sequence
  misc_feature 1..13: note = U can be replaced by T. Any base can be replaced with a modified base.
  source 1..13: mol_type = other RNA
cgccgggggtcag

SEQ ID NO: 531 - RNA, 13 nt, synthetic construct
  misc_feature 1..13: note = Synthetic sequence
  misc_feature 1..13: note = U can be replaced by T. Any base can be replaced with a modified base.
  source 1..13: mol_type = other RNA
tcgccgggggtca

SEQ ID NO: 532 - RNA, 13 nt, synthetic construct
  misc_feature 1..13: note = Synthetic sequence
  misc_feature 1..13: note = U can be replaced by T. Any base can be replaced with a modified base.
  source 1..13: mol_type = other RNA
gtcgccgggggtc

SEQ ID NO: 533 - RNA, 13 nt, synthetic construct
  misc_feature 1..13: note = Synthetic sequence
  misc_feature 1..13: note = U can be replaced by T. Any base can be replaced with a modified base.
  source 1..13: mol_type = other RNA
ggtcgccgggggt

SEQ ID NO: 534 - RNA, 13 nt, synthetic construct
  misc_feature 1..13: note = Synthetic sequence
  misc_feature 1..13: note = U can be replaced by T. Any base can be replaced with a modified base.
  source 1..13: mol_type = other RNA
gggtcgccggggg

SEQ ID NO: 535 - RNA, 13 nt, synthetic construct
  misc_feature 1..13: note = Synthetic sequence
  misc_feature 1..13: note = U can be replaced by T. Any base can be replaced with a modified base.
  source 1..13: mol_type = other RNA
ggggtcgccgggg

SEQ ID NO: 536 - RNA, 13 nt, synthetic construct
  misc_feature 1..13: note = Synthetic sequence
  misc_feature 1..13: note = U can be replaced by T. Any base can be replaced with a modified base.
  source 1..13: mol_type = other RNA
aggggtcgccggg

SEQ ID NO: 537 - RNA, 13 nt, synthetic construct
  misc_feature 1..13: note = Synthetic sequence
  misc_feature 1..13: note = U can be replaced by T. Any base can be replaced with a modified base.
  source 1..13: mol_type = other RNA
aaggggtcgccgg

SEQ ID NO: 538 - RNA, 13 nt, synthetic construct
  misc_feature 1..13: note = Synthetic sequence
  misc_feature 1..13: note = U can be replaced by T. Any base can be replaced with a modified base.
  source 1..13: mol_type = other RNA
caaggggtcgccg

SEQ ID NO: 539 - RNA, 13 nt, synthetic construct
  misc_feature 1..13: note = Synthetic sequence
  misc_feature 1..13: note = U can be replaced by T. Any base can be replaced with a modified base.
  source 1..13: mol_type = other RNA
gcaaggggtcgcc

SEQ ID NO: 540 - RNA, 13 nt, synthetic construct
  misc_feature 1..13: note = Synthetic sequence
  misc_feature 1..13: note = U can be replaced by T. Any base can be replaced with a modified base.
  source 1..13: mol_type = other RNA
tgcaaggggtcgc

SEQ ID NO: 541 - RNA, 13 nt, synthetic construct
  misc_feature 1..13: note = Synthetic sequence
  misc_feature 1..13: note = U can be replaced by T. Any base can be replaced with a modified base.
  source 1..13: mol_type = other RNA
gtgcaaggggtcg

SEQ ID NO: 542 - RNA, 13 nt, synthetic construct
  misc_feature 1..13: note = Synthetic sequence
  misc_feature 1..13: note = U can be replaced by T. Any base can be replaced with a modified base.
  source 1..13: mol_type = other RNA
agtgcaaggggtc

SEQ ID NO: 543 - RNA, 13 nt, synthetic construct
  misc_feature 1..13: note = Synthetic sequence
  misc_feature 1..13: note = U can be replaced by T. Any base can be replaced with a modified base.
  source 1..13: mol_type = other RNA
gagtgcaaggggt

SEQ ID NO: 544 - RNA, 13 nt, synthetic construct
  misc_feature 1..13: note = Synthetic sequence
  misc_feature 1..13: note = U can be replaced by T. Any base can be replaced with a modified base.
  source 1..13: mol_type = other RNA
agagtgcaagggg

SEQ ID NO: 545 - RNA, 13 nt, synthetic construct
  misc_feature 1..13: note = Synthetic sequence
  misc_feature 1..13: note = U can be replaced by T. Any base can be replaced with a modified base.
  source 1..13: mol_type = other RNA
gagagtgcaaggg

SEQ ID NO: 546 - RNA, 13 nt, synthetic construct
  misc_feature 1..13: note = Synthetic sequence
  misc_feature 1..13: note = U can be replaced by T. Any base can be replaced with a modified base.
  source 1..13: mol_type = other RNA
ggagagtgcaagg

SEQ ID NO: 547 - RNA, 80 nt, Homo sapiens
  source 1..80: mol_type = other RNA
atgagtagataaaaggatggatggagagatgggtgagtacatggatggatagatggatgagttggtgggtagattcgtgc

SEQ ID NO: 548 - RNA, 80 nt, Homo sapiens
  source 1..80: mol_type = other RNA
atgagtagataaaagcatggatggagagatgggtgagtacatggatggatagatggatgagttggtgggtagattcgtgc

SEQ ID NO: 549 - RNA, 40 nt, Homo sapiens
  source 1..40: mol_type = other RNA
ggatggatggagagatgggtgagtacatggatggatagat

SEQ ID NO: 550 - RNA, 40 nt, Homo sapiens
  source 1..40: mol_type = other RNA
gcatggatggagagatgggtgagtacatggatggatagat

SEQ ID NO: 551 - RNA, 29 nt, Homo sapiens
  source 1..29: mol_type = other RNA
atggagagatgggtgagtacatggatgga

SEQ ID NO: 552 - RNA, 97 nt, Homo sapiens
  source 1..97: mol_type = other RNA
gttcttccttctattccagccctaaccactcaggattgggccgtttgtgtctgggtatgtctcttccagctgcctgggtttcctggaaagaactctt

SEQ ID NO: 553 - RNA, 43 nt, Homo sapiens
  source 1..43: mol_type = other RNA
gtgtctgggtatgtctcttccagctgcctgggtttcctggaaa

SEQ ID NO: 554 - RNA, 46 nt, Homo sapiens
  source 1..46: mol_type = other RNA
tcatcaggttcttccttctattccagccctaaccactcaggattgg

SEQ ID NO: 555 - DNA, 21 bp, synthetic construct
  modified_base 1..21: mod_base = OTHER; note = * = a phosphorothioate, + = LNA
  modified_base 1..21: mod_base = OTHER; note = phosphorothioate linkage, LNA at positions 1, 4, 7, 10, 13, 16, 19
  source 1..21: mol_type = other DNA
cacccatctctccatccatgc

SEQ ID NO: 556 - DNA, 21 bp, synthetic construct
  misc_feature 1..21: note = Synthetic sequence
  modified_base 1..21: mod_base = OTHER; note = phosphorthioate backbone, and LNA at positions 1, 4, 7, 10, 13, 16 and 19
  modified_base 1..21: mod_base = OTHER; note = phosphorthioate linkage, and LNA at positions 1, 4, 7, 10, 13, 16 and 19
  source 1..21: mol_type = other DNA
cacccatctctccatccatcc

SEQ ID NO: 557 - DNA, 21 bp, synthetic construct
  misc_feature 1..21: note = Synthetic sequence
  modified_base 1..21: mod_base = OTHER; note = phosphorthioate backbone, LNA at positions 1, 4, 7, 10, 13, 16, 19 and 21
  modified_base 1..21: mod_base = OTHER; note = phosphorthioate linkage, LNA at positions 1, 4, 7, 10, 13, 16, 19 and 21
  source 1..21: mol_type = other DNA
ctcacccatctctccatccat

SEQ ID NO: 558 - DNA, 21 bp, synthetic construct
  misc_feature 1..21: note = Synthetic sequence
  modified_base 1..21: mod_base = OTHER; note = phosphorthioate backbone, LNA at positions 1, 4, 7, 10, 13, 16, 19 and 21
  modified_base 1..21: mod_base = OTHER; note = phosphorthioate linkage, LNA at positions 1, 4, 7, 10, 13, 16, 19 and 21
  source 1..21: mol_type = other DNA
tgtactcacccatctctccat

SEQ ID NO: 559 - DNA, 21 bp, synthetic construct
  misc_feature 1..21: note = Synthetic sequence
  modified_base 1..21: mod_base = OTHER; note = phosphorthioate backbone, LNA at positions 1, 4, 7, 10, 13, 16, 19 and 21
  modified_base 1..21: mod_base = OTHER; note = phosphorthioate linkage, LNA at positions 1, 4, 7, 10, 13, 16, 19 and 21
  source 1..21: mol_type = other DNA
tccatgtactcacccatctct

SEQ ID NO: 560 - DNA, 21 bp, synthetic construct
  misc_feature 1..21: note = Synthetic sequence
  modified_base 1..21: mod_base = OTHER; note = phosphorthioate backbone, LNA at positions 1, 4, 7, 10, 13, 16, 19 and 21
  modified_base 1..21: mod_base = OTHER; note = phosphorthioate linkage, LNA at positions 1, 4, 7, 10, 13, 16, 19 and 21
  source 1..21: mol_type = other DNA
tccatccatgtactcacccat

SEQ ID NO: 561 - DNA, 21 bp, synthetic construct
  misc_feature 1..21: note = Synthetic sequence
  modified_base 1..21: mod_base = OTHER; note = phosphorthioate backbone, LNA at positions 1, 4, 7, 10, 13, 16, 19 and 21
  modified_base 1..21: mod_base = OTHER; note = phosphorthioate linkage, LNA at positions 1, 4, 7, 10, 13, 16, 19 and 21
  source 1..21: mol_type = other DNA
atctatccatccatgtactca

SEQ ID NO: 562 - DNA, 17 bp, synthetic construct
  misc_feature 1..17: note = Synthetic sequence
  modified_base 1..17: mod_base = OTHER; note = phosphorthioate backbone, LNA at postions 1, 4, 7, 10, 13, 16 and 17
  modified_base 1..17: mod_base = OTHER; note = phosphorthioate linkage, LNA at postions 1, 4, 7, 10, 13, 16 and 17
  source 1..17: mol_type = other DNA
tcacccatctctccatc

SEQ ID NO: 563 - DNA, 17 bp, synthetic construct
  misc_feature 1..17: note = Synthetic sequence
  modified_base 1..17: mod_base = OTHER; note = phosphorothioate linkage, LNA at 1, 3, 5, 7, 9, 11, 13, 15 and 17
  source 1..17: mol_type = other DNA
tcacccatctctccatc

SEQ ID NO: 564 - DNA, 17 bp, synthetic construct
  misc_feature 1..17: note = Synthetic sequence
  modified_base 1..17: mod_base = OTHER; note = phosphorthioate backbone, LNA bases at 1, 4, 7, 10, 13, 16 and 17
  modified_base 1..17: mod_base = OTHER; note = phosphorothioate linkage, LNA bases at 1, 4, 7, 10, 13, 16 and 17
  source 1..17: mol_type = other DNA
gtactcacccatctctc

SEQ ID NO: 565 - DNA, 17 bp, synthetic construct
  misc_feature 1..17: note = Synthetic sequence
  modified_base 1..17: mod_base = OTHER; note = phosphorthioate backbone, LNA at positins 1, 3, 5, 7, 9, 11, 13, 15 and 17
  source 1..17: mol_type = other DNA
gtactcacccatctctc

SEQ ID NO: 566 - DNA, 13 bp, synthetic construct
  misc_feature 1..13: note = Synthetic sequence
  modified_base 1..13: mod_base = OTHER; note = phosphorthioate backbone, LNA bases at 2, 4, 6, 8, 10 and 12
  modified_base 1..13: mod_base = OTHER; note = phosphorthioate linkage, LNA bases at 2, 4, 6, 8, 10 and 12
  source 1..13: mol_type = other DNA
cacccatctctcc

SEQ ID NO: 567 - RNA, 25 nt, synthetic construct
  misc_feature 1..25: note = Synthetic sequence
  modified_base 1..25: mod_base = OTHER; note = phosphorthioate backbone and 2-OMe-RNA at all positions
  modified_base 1..25: mod_base = OTHER; note = phosphorthioate linkage and 2-OMe-RNA at all positions
  source 1..25: mol_type = other RNA
catgtactcacccatctctccatcc

SEQ ID NO: 568 - RNA, 30 nt, synthetic construct
  misc_feature 1..30: note = Synthetic sequence
  modified_base 1..30: mod_base = OTHER; note = phosphorthioate backbone, all bases substitued with 2--O-methyl-RNA
  modified_base 1..30: mod_base = OTHER; note = phosphorthioate linkage, all bases substitued with 2--O-methyl-RNA
  source 1..30: mol_type = other RNA
atccatgtactcacccatctctccatccat

SEQ ID NO: 569 - DNA, 21 bp, synthetic construct
  misc_feature 1..21: note = Synthetic sequence
  modified_base 1..21: mod_base = OTHER; note = phosphorthioate backbone, LNA at positions 1, 4, 7, 10, 13, 16, 19 and 21
  modified_base 1..21: mod_base = OTHER; note = phosphorthioate linkage, LNA at positions 1, 4, 7, 10, 13, 16, 19 and 21
  source 1..21: mol_type = other DNA
caggcagctggaagagacata

SEQ ID NO: 570 - DNA, 21 bp, synthetic construct
  misc_feature 1..21: note = Synthetic sequence
  modified_base 1..21: mod_base = OTHER; note = phosphorothioate linkage, LNA at positions 2, 4, 7, 10, 13, 16, 19 and 21
  source 1..21: mol_type = other DNA
aacccaggcagctggaagaga

SEQ ID NO: 571 - DNA, 21 bp, synthetic construct
  misc_feature 1..21: note = Synthetic sequence
  modified_base 1..21: mod_base = OTHER; note = phosphorthioate backbone, LNA at positions 1, 4, 7, 10, 13, 16, 19 and 21
  modified_base 1..21: mod_base = OTHER; note = phosphorthioate linkage, LNA at positions 1, 4, 7, 10, 13, 16, 19 and 21
  source 1..21: mol_type = other DNA
ggaaacccaggcagctggaag

SEQ ID NO: 572 - DNA, 13 bp, synthetic construct
  misc_feature 1..13: note = Synthetic sequence
  source 1..13: mol_type = other DNA
agttttcaattcc

SEQ ID NO: 573 - DNA, 20 bp, synthetic construct
  misc_feature 1..20: note = Synthetic sequence
  source 1..20: mol_type = other DNA
gacatcaaatcccgcgtgaa

SEQ ID NO: 574 - DNA, 20 bp, synthetic construct
  misc_feature 1..20: note = Synthetic sequence
  source 1..20: mol_type = other DNA
cattgatgttggcgagcagg

SEQ ID NO: 575 - DNA, 20 bp, synthetic construct
  misc_feature 1..20: note = Synthetic sequence
  source 1..20: mol_type = other DNA
cagacgatcattgaggtgcg

SEQ ID NO: 576 - DNA, 20 bp, synthetic construct
  misc_feature 1..20: note = Synthetic sequence
  source 1..20: mol_type = other DNA
atacttggaggagaggcagg

SEQ ID NO: 577 - DNA, 18 bp, synthetic construct
  misc_feature 1..18: note = Synthetic sequence
  source 1..18: mol_type = other DNA
caagcgaactgacaaatc

SEQ ID NO: 578 - DNA, 17 bp, synthetic construct
  misc_feature 1..17: note = Synthetic sequence
  source 1..17: mol_type = other DNA
ctgggatcttcacgacc

SEQ ID NO: 579 - DNA, 21 bp, synthetic construct
  misc_feature 1..21: note = Synthetic sequence
  modified_base 1..21: mod_base = OTHER; note = phosphorothioate linkage, LNA at bases 1, 4, 7, 10, 13, 16, 19, and 21
  source 1..21: mol_type = other DNA
tagggctggaatagaaggaag

SEQ ID NO: 580 - DNA, 21 bp, synthetic construct
  misc_feature 1..21: note = Synthetic sequence
  modified_base 1..21: mod_base = OTHER; note = phosphorothioate linkage, LNA at bases 1, 4, 7, 10, 13, 16, 19, and 21
  source 1..21: mol_type = other DNA
tgagtggttagggctggaata

SEQ ID NO: 581 - RNA, 65 nt, synthetic construct
  source 1..65: mol_type = other RNA
aaaagcatggatggagagatgggtgaggaaaaatggatgggtggataaattgatgggtggatgga

SEQ ID NO: 582 - RNA, 35 nt, synthetic construct
  source 1..35: mol_type = other RNA
taaaaggaaaaggaaggatggggatggagatggat

SEQ ID NO: 583 - RNA, 35 nt, synthetic construct
  source 1..35: mol_type = other RNA
taaaagcaaaagcaagcatgggcatggacatggat